European Patent Specification EP 3 464 383 B1, published July 31, 2024. Title: REVERSAL BINDING AGENTS FOR ANTI-FACTOR XI/XIA ANTIBODIES AND USES THEREOF. Applicant: NOVARTIS AG. The sequence listing filed with the application follows.

SEQUENCE LISTING (394 sequences)

SEQ ID NO: 1 - protein, 625 aa, Homo sapiens [sequence omitted]

SEQ ID NO: 2 - DNA, 3278 bp, Homo sapiens
aggcacacaggcaaaatcaagttctacatctgtccctgtgtatgtcacttgtttgaatacgaaataaaattaaaaaaataaattcagtgtattgagaaagcaagcaattctctcaaggtatatttctgacatactaagattttaacgactttcacaaatatgctgtactgagagagaatgttacataacattgagaactagtacaagtaaatattaaagtgaagtgaccatttcctacacaagctcattcagaggaggatgaagaccattttggaggaagaaaagcacccttattaagaattgcagcaagtaagccaacaaggtcttttcaggatgattttcttatatcaagtggtacatttcattttatttacttcagtttctggtgaatgtgtgactcagttgttgaaggacacctgctttgaaggaggggacattactacggtcttcacaccaagcgccaagtactgccaggtagtctgcacttaccacccaagatgtttactcttcactttcacggcggaatcaccatctgaggatcccacccgatggtttacttgtgtcctgaaagacagtgttacagaaacactgccaagagtgaataggacagcagcgatttctgggtattctttcaagcaatgctcacaccaaataagcgcttgcaacaaagacatttatgtggacctagacatgaagggcataaactataacagctcagttgccaagagtgctcaagaatgccaagaaagatgcacggatgacgtccactgccactttttcacgtacgccacaaggcagtttcccagcctggagcatcgtaacatttgtctactgaagcacacccaaacagggacaccaaccagaataacgaagctcgataaagtggtgtctggattttcactgaaatcctgtgcactttctaatctggcttgtattagggacattttccctaatacggtgtttgcagacagcaacatcgacagtgtcatggctcccgatgcttttgtctgtggccgaatctgcactcatcatcccggttgcttgttttttaccttcttttcccaggaatggcccaaagaatctcaaagaaatctttgtctccttaaaacatctgagagtggattgcccagtacacgcattaaaaagagcaaagctctttctggtttcagtctacaaagctgcaggcacagcatcccagtgttctgccattcttcattttaccatgacactgatttcttgggagaagaactggatattgttgctgcaaaaagtcacgaggcctgccagaaactgtgcaccaatgccgtccgctgccagttttttacctataccccagcccaagcatcctgcaacgaagggaagggcaagtgttacttaaagctttcttcaaacggatctccaactaaaatacttcacgggagaggaggcatctctggatacacattaaggttgtgtaaaatggataatgagtgtaccaccaaaatcaagcccaggatcgttggaggaactgcgtctgttcgtggtgagtggccgtggcaggtgaccctgcacacaacctcacccactcagagacacctgtgtggaggctccatcattggaaaccagtggatattaacagccgctcactgtttctatggggtagagtcacctaagattttgcgtgtctacagtggcattttaaatcaatctgaaataaaagaggacacatctttctttggggttcaagaaataataatccatgatcagtataaaatggcagaaagcgggtatgatattgccttgttgaaactggaaaccacagtgaattacacagattctcaacgacccatatgcctgccttccaaaggagatagaaatgtaatatacactgattgctgggtgactggatgggggtacagaaaactaagagacaaaatacaaaatactctccagaaagccaagatacccttagtgaccaacgaagagtgccagaagagatacagaggacataaaataacccataagatgatctgtgccggctacagggaaggagggaaggacgcttgcaagggagattcgggaggccctctgtcctgcaaacacaatgaggtctggcatctggtaggcatcacgagctggggcgaaggctgtgctcaaagggagcggccaggtgtttacaccaacgtggtcgagtacgtggactggattctggagaaaactcaagcagtgtgaatgggttcccaggggccattggagtccctgaaggacccaggatttgctgggagagggtgttgagttcactgtgccagcatgcttcctccacagtaacacgctgaaggggcttggtgtttgtaagaaaatgctagaagaaaacaaactgtcacaagttgttatgtccaaaactcccgttctatgatcgttgtagtttgtttgagcattcagtctctttgtttttgatcacgcttctatggagtccaagaattaccataaggcaatatttctgaagattactatataggcagatatagcagaaaataaccaagtagtggcagtggggatcaggcagaagaactggtaaaagaagccaccataaatagatttgttcgatgaaagatgaaaactggaagaaaggagaacaaagacagtcttcaccattttgcaggaatctacactctgcctatgtgaacacatttcttttgtaaagaaagaaattgattgcatttaatggcagattttcagaatagtcaggaattcttgtcatttccattttaaaatatatattaaaaaaaatcagttcgagtagacacgagctaagagtgaatgtgaagataacagaatttctgtgtggaagaggattacaagcagcaatttacctggaagtgataccttaggggcaatcttgaagatacactttcctgaaaaatgatttgtgatggattgtatatttatttaaaatatcttgggaggggaggctgatggagatagggagcatgctcaaacctccctaagacaagctgctgctgtgactatgggctcccaaagagctagatcgtatatttatttgacaaaaatcaccatagactgcatccatactacagagaaaaaacaattagggcgcaaatggatagttacagtaaagtcttcagcaagcagctgcctgtattctaagcactgggattttctgtttcgtgcaaatatttatctcattattgttgtgatctagttcaataacctagaatttgaattgtcaccacatagctttcaatctgtgccaacaactatacaattcatcaagtgtg

SEQ ID NO: 3 - protein, 10 aa, Artificial Sequence
  source: /note="Description of Artificial Sequence: Synthetic peptide"
GFTFSTAAMS

SEQ ID NO: 4 - protein, 17 aa, Artificial Sequence
  source: /note="Description of Artificial Sequence: Synthetic peptide"
GISGSGSSTYYADSVKG

SEQ ID NO: 5 - protein, 13 aa, Artificial Sequence
  source: /note="Description of Artificial Sequence: Synthetic peptide"
ELSYLYSGYYFDY

SEQ ID NO: 6 - protein, 5 aa, Artificial Sequence
  source: /note="Description of Artificial Sequence: Synthetic peptide"
TAAMS

SEQ ID NO: 7 - protein, 7 aa, Artificial Sequence
  source: /note="Description of Artificial Sequence: Synthetic peptide"
GFTFSTA

SEQ ID NO: 8 - protein, 6 aa, Artificial Sequence
  source: /note="Description of Artificial Sequence: Synthetic peptide"
SGSGSS

SEQ ID NO: 9 - protein, 8 aa, Artificial Sequence
  source: /note="Description of Artificial Sequence: Synthetic peptide"
GFTFSTAA

SEQ ID NO: 10 - protein, 8 aa, Artificial Sequence
  source: /note="Description of Artificial Sequence: Synthetic peptide"
ISGSGSST

SEQ ID NO: 11 - protein, 15 aa, Artificial Sequence
  source: /note="Description of Artificial Sequence: Synthetic peptide"
ARELSYLYSGYYFDY

SEQ ID NO: 12 - protein, 122 aa, Artificial Sequence
  source: /note="Description of Artificial Sequence: Synthetic polypeptide"
QVQLLESGGGLVQPGGSLRLSCAASGFTFSTAAMSWVRQAPGKGLEWVSGISGSGSSTYYADSVKGRFTISRDNSKNTLYLQMNSLRAEDTAVYYCARELSYLYSGYYFDYWGQGTLVTVSS

SEQ ID NO: 13 - DNA, 366 bp, Artificial Sequence
  source: /note="Description of Artificial Sequence: Synthetic polynucleotide"
caggtgcagctgctggaatcaggcggcggactggtgcagcctggcggtagcctgagactgagctgcgctgctagtggcttcacctttagcaccgccgctatgagctgggttcgacaggccccagggaaaggcctcgagtgggtctcagggattagcggtagcggctctagcacctactacgccgatagcgtgaagggccggttcactatctctagggataactctaagaacaccctgtacctgcagatgaatagcctgagagccgaggacaccgccgtctactactgcgctagagagctgagctacctgtatagcggctactacttcgactactggggtcaaggcaccctggtcaccgtgtctagc

SEQ ID NO: 14 - protein, 452 aa, Artificial Sequence
  source: /note="Description of Artificial Sequence: Synthetic polypeptide"
QVQLLESGGGLVQPGGSLRLSCAASGFTFSTAAMSWVRQAPGKGLEWVSGISGSGSSTYYADSVKGRFTISRDNSKNTLYLQMNSLRAEDTAVYYCARELSYLYSGYYFDYWGQGTLVTVSSASTKGPSVFPLAPSSKSTSGGTAALGCLVKDYFPEPVTVSWNSGALTSGVHTFPAVLQSSGLYSLSSVVTVPSSSLGTQTYICNVNHKPSNTKVDKRVEPKSCDKTHTCPPCPAPELLGGPSVFLFPPKPKDTLMISRTPEVTCVVVAVSHEDPEVKFNWYVDGVEVHNAKTKPREEQYNSTYRVVSVLTVLHQDWLNGKEYKCKVSNKALAAPIEKTISKAKGQPREPQVYTLPPSREEMTKNQVSLTCLVKGFYPSDIAVEWESNGQPENNYKTTPPVLDSDGSFFLYSKLTVDKSRWQQGNVFSCSVMHEALHNHYTQKSLSLSPGK

SEQ ID NO: 15 - DNA, 1356 bp, Artificial Sequence
  source: /note="Description of Artificial Sequence: Synthetic polynucleotide"
caggtgcagctgctggaatcaggcggcggactggtgcagcctggcggtagcctgagactgagctgcgctgctagtggcttcacctttagcaccgccgctatgagctgggttcgacaggccccagggaaaggcctcgagtgggtctcagggattagcggtagcggctctagcacctactacgccgatagcgtgaagggccggttcactatctctagggataactctaagaacaccctgtacctgcagatgaatagcctgagagccgaggacaccgccgtctactactgcgctagagagctgagctacctgtatagcggctactacttcgactactggggtcaaggcaccctggtcaccgtgtctagcgctagcactaagggcccctccgtgttccctctggccccttccagcaagtctacctccggcggcacagctgctctgggctgcctggtcaaggactacttccctgagcctgtgacagtgtcctggaactctggcgccctgacctctggcgtgcacaccttccctgccgtgctgcagtcctccggcctgtactccctgtcctccgtggtcacagtgccttcaagcagcctgggcacccagacctatatctgcaacgtgaaccacaagccttccaacaccaaggtggacaagcgggtggagcctaagtcctgcgacaagacccacacctgtcctccctgccctgctcctgaactgctgggcggcccttctgtgttcctgttccctccaaagcccaaggacaccctgatgatctcccggacccctgaagtgacctgcgtggtggtggccgtgtcccacgaggatcctgaagtgaagttcaattggtacgtggacggcgtggaggtgcacaacgccaagaccaagcctcgggaggaacagtacaactccacctaccgggtggtgtccgtgctgaccgtgctgcaccaggactggctgaacggcaaagagtacaagtgcaaagtctccaacaaggccctggccgcccctatcgaaaagacaatctccaaggccaagggccagcctagggaaccccaggtgtacaccctgccacccagccgggaggaaatgaccaagaaccaggtgtccctgacctgtctggtcaagggcttctacccttccgatatcgccgtggagtgggagtctaacggccagcctgagaacaactacaagaccacccctcctgtgctggactccgacggctccttcttcctgtactccaaactgaccgtggacaagtcccggtggcagcagggcaacgtgttctcctgctccgtgatgcacgaggccctgcacaaccactacacccagaagtccctgtccctgtctcccggcaag

SEQ ID NO: 16 - protein, 13 aa, Artificial Sequence
  source: /note="Description of Artificial Sequence: Synthetic peptide"
SGSSSNIGSNDVS

SEQ ID NO: 17 - protein, 7 aa, Artificial Sequence
  source: /note="Description of Artificial Sequence: Synthetic peptide"
KNYNRPS

SEQ ID NO: 18 - protein, 11 aa, Artificial Sequence
  source: /note="Description of Artificial Sequence: Synthetic peptide"
SAWDQRQFDVV

SEQ ID NO: 19 - protein, 9 aa, Artificial Sequence
  source: /note="Description of Artificial Sequence: Synthetic peptide"
SSSNIGSND

SEQ ID NO: 20 - protein, 3 aa, Artificial Sequence
  source: /note="Description of Artificial Sequence: Synthetic peptide"
KNY

SEQ ID NO: 21 - protein, 8 aa, Artificial Sequence
  source: /note="Description of Artificial Sequence: Synthetic peptide"
WDQRQFDV

SEQ ID NO: 22 - protein, 8 aa, Artificial Sequence
  source: /note="Description of Artificial Sequence: Synthetic peptide"
SSNIGSND

SEQ ID NO: 23 - protein, 110 aa, Artificial Sequence
  source: /note="Description of Artificial Sequence: Synthetic polypeptide"
QSVLTQPPSASGTPGQRVTISCSGSSSNIGSNDVSWYQQLPGTAPKLLIYKNYNRPSGVPDRFSGSKSGTSASLAISGLQSEDEADYYCSAWDQRQFDVVFGGGTKLTVL

SEQ ID NO: 24 - DNA, 330 bp, Artificial Sequence
  source: /note="Description of Artificial Sequence: Synthetic polynucleotide"
cagtcagtcctgactcagccccctagcgctagtggcacccctggtcaaagagtgactattagctgtagcggctctagctctaatatcggctctaacgacgtcagctggtatcagcagctgcccggcaccgcccctaagctgctgatctataagaactataataggcctagcggcgtgcccgataggtttagcggatctaaatcagggacttctgctagtctggctattagcggcctgcagtcagaggacgaggccgactactactgtagcgcctgggatcagcgtcagttcgacgtggtgttcggcggaggcactaagctgaccgtgctg

SEQ ID NO: 25 - protein, 216 aa, Artificial Sequence
  source: /note="Description of Artificial Sequence: Synthetic polypeptide"
QSVLTQPPSASGTPGQRVTISCSGSSSNIGSNDVSWYQQLPGTAPKLLIYKNYNRPSGVPDRFSGSKSGTSASLAISGLQSEDEADYYCSAWDQRQFDVVFGGGTKLTVLGQPKAAPSVTLFPPSSEELQANKATLVCLISDFYPGAVTVAWKADSSPVKAGVETTTPSKQSNNKYAASSYLSLTPEQWKSHRSYSCQVTHEGSTVEKTVAPTECS

SEQ ID NO: 26 - DNA, 648 bp, Artificial Sequence
  source: /note="Description of Artificial Sequence: Synthetic polynucleotide"
cagtcagtcctgactcagccccctagcgctagtggcacccctggtcaaagagtgactattagctgtagcggctctagctctaatatcggctctaacgacgtcagctggtatcagcagctgcccggcaccgcccctaagctgctgatctataagaactataataggcctagcggcgtgcccgataggtttagcggatctaaatcagggacttctgctagtctggctattagcggcctgcagtcagaggacgaggccgactactactgtagcgcctgggatcagcgtcagttcgacgtggtgttcggcggaggcactaagctgaccgtgctgggtcaacctaaggctgcccccagcgtgaccctgttcccccccagcagcgaggagctgcaggccaacaaggccaccctggtgtgcctgatcagcgacttctacccaggcgccgtgaccgtggcctggaaggccgacagcagccccgtgaaggccggcgtggagaccaccacccccagcaagcagagcaacaacaagtacgccgccagcagctacctgagcctgacccccgagcagtggaagagccacaggtcctacagctgccaggtgacccacgagggcagcaccgtggaaaagaccgtggccccaaccgagtgcagc

SEQ ID NO: 27 - protein, 10 aa, Artificial Sequence
  source: /note="Description of Artificial Sequence: Synthetic peptide"
GFTFSDYAMS

SEQ ID NO: 28 - protein, 17 aa, Artificial Sequence
  source: /note="Description of Artificial Sequence: Synthetic peptide"
VIDYSSSNTYYADSVKG

SEQ ID NO: 29 - protein, 12 aa, Artificial Sequence
  source: /note="Description of Artificial Sequence: Synthetic peptide"
EGYSYRSIRFDY

SEQ ID NO: 30 - protein, 5 aa, Artificial Sequence
  source: /note="Description of Artificial Sequence: Synthetic peptide"
DYAMS

SEQ ID NO: 31 - protein, 17 aa, Artificial Sequence
  source: /note="Description of Artificial Sequence: Synthetic peptide"
VIDYSSSNTYYADSVKG

SEQ ID NO: 32 - protein, 12 aa, Artificial Sequence
  source: /note="Description of Artificial Sequence: Synthetic peptide"
EGYSYRSIRFDY

SEQ ID NO: 33 - protein, 7 aa, Artificial Sequence
  source: /note="Description of Artificial Sequence: Synthetic peptide"
GFTFSDY

SEQ ID NO: 34 - protein, 6 aa, Artificial Sequence
  source: /note="Description of Artificial Sequence: Synthetic peptide"
DYSSSN

SEQ ID NO: 35 - protein, 12 aa, Artificial Sequence
  source: /note="Description of Artificial Sequence: Synthetic peptide"
EGYSYRSIRFDY

SEQ ID NO: 36 - protein, 8 aa, Artificial Sequence
  source: /note="Description of Artificial Sequence: Synthetic peptide"
GFTFSDYA

SEQ ID NO: 37 - protein, 8 aa, Artificial Sequence
  source: /note="Description of Artificial Sequence: Synthetic peptide"
IDYSSSNT

SEQ ID NO: 38 - protein, 14 aa, Artificial Sequence
  source: /note="Description of Artificial Sequence: Synthetic peptide"
AREGYSYRSIRFDY

SEQ ID NO: 39 - protein, 121 aa, Artificial Sequence
  source: /note="Description of Artificial Sequence: Synthetic polypeptide"
QVQLLESGGGLVQPGGSLRLSCAASGFTFSDYAMSWVRQAPGKGLEWVSVIDYSSSNTYYADSVKGRFTISRDNSKNTLYLQMNSLRAEDTAVYYCAREGYSYRSIRFDYWGQGTLVTVSS

SEQ ID NO: 40 - DNA, 363 bp, Artificial Sequence
  source: /note="Description of Artificial Sequence: Synthetic polynucleotide"
caagtgcagctgctggaatctggcggcggactggtgcagcctggcggtagtctgagactgtcttgcgccgcctccggcttcaccttctccgactacgccatgtcctgggtccgacaggcccctggcaagggcctggagtgggtgtccgtgatcgactactcctcctccaacacctactacgccgactccgtgaagggccggttcaccatctcccgggacaactccaagaacaccctgtacctgcagatgaactccctgcgggccgaggacaccgccgtgtactactgcgccagagagggctactcctaccggtccatcagattcgactactggggccagggcaccctggtcaccgtgtcctct

SEQ ID NO: 41 - protein, 224 aa, Artificial Sequence
  source: /note="Description of Artificial Sequence: Synthetic polypeptide"
QVQLLESGGGLVQPGGSLRLSCAASGFTFSDYAMSWVRQAPGKGLEWVSVIDYSSSNTYYADSVKGRFTISRDNSKNTLYLQMNSLRAEDTAVYYCAREGYSYRSIRFDYWGQGTLVTVSSASTKGPSVFPLAPSSKSTSGGTAALGCLVKDYFPEPVTVSWNSGALTSGVHTFPAVLQSSGLYSLSSVVTVPSSSLGTQTYICNVNHKPSNTKVDKRVEPKSC

SEQ ID NO: 42 - DNA, 672 bp, Artificial Sequence
  source: /note="Description of Artificial Sequence: Synthetic polynucleotide"
caagtgcagctgctggaatctggcggcggactggtgcagcctggcggtagtctgagactgtcttgcgccgcctccggcttcaccttctccgactacgccatgtcctgggtccgacaggcccctggcaagggcctggagtgggtgtccgtgatcgactactcctcctccaacacctactacgccgactccgtgaagggccggttcaccatctcccgggacaactccaagaacaccctgtacctgcagatgaactccctgcgggccgaggacaccgccgtgtactactgcgccagagagggctactcctaccggtccatcagattcgactactggggccagggcaccctggtcaccgtgtcctctgctagcaccaagggcccctccgtgttccctctggccccttccagcaagtctacctctggcggcaccgctgctctgggctgcctggtgaaggactacttccctgagcctgtgacagtgtcctggaactctggcgccctgacctccggcgtgcacaccttccctgccgtgctgcagtcctccggcctgtactccctgtcctccgtggtgacagtgccttcctccagcctgggcacccagacctatatctgcaacgtgaaccacaagccttccaacaccaaggtggacaagcgggtggagcctaagtcatgc

SEQ ID NO: 43 - protein, 11 aa, Artificial Sequence
  source: /note="Description of Artificial Sequence: Synthetic peptide"
RASQSISSNLN

SEQ ID NO: 44 - protein, 7 aa, Artificial Sequence
  source: /note="Description of Artificial Sequence: Synthetic peptide"
AASNLQS

SEQ ID NO: 45 - protein, 9 aa, Artificial Sequence
  source: /note="Description of Artificial Sequence: Synthetic peptide"
LQFDHTPFT

SEQ ID NO: 46 - protein, 11 aa, Artificial Sequence
  source: /note="Description of Artificial Sequence: Synthetic peptide"
RASQSISSNLN

SEQ ID NO: 47 - protein, 7 aa, Artificial Sequence
  source: /note="Description of Artificial Sequence: Synthetic peptide"
AASNLQS

SEQ ID NO: 48 - protein, 9 aa, Artificial Sequence
  source: /note="Description of Artificial Sequence: Synthetic peptide"
LQFDHTPFT

SEQ ID NO: 49 - protein, 7 aa, Artificial Sequence
  source: /note="Description of Artificial Sequence: Synthetic peptide"
SQSISSN

SEQ ID NO: 50 - protein, 3 aa, Artificial Sequence
  source: /note="Description of Artificial Sequence: Synthetic peptide"
AAS

SEQ ID NO: 51 - protein, 6 aa, Artificial Sequence
  source: /note="Description of Artificial Sequence: Synthetic peptide"
FDHTPF

SEQ ID NO: 52 - protein, 6 aa, Artificial Sequence
  source: /note="Description of Artificial Sequence: Synthetic peptide"
QSISSN

SEQ ID NO: 53 - protein, 3 aa, Artificial Sequence
  source: /note="Description of Artificial Sequence: Synthetic peptide"
AAS

SEQ ID NO: 54 - protein, 9 aa, Artificial Sequence
  source: /note="Description of Artificial Sequence: Synthetic peptide"
LQFDHTPFT

SEQ ID NO: 55 - protein, 107 aa, Artificial Sequence
  source: /note="Description of Artificial Sequence: Synthetic polypeptide"
DIQMTQSPSSLSASVGDRVTITCRASQSISSNLNWYQQKPGKAPKLLIYAASNLQSGVPSRFSGSGSGTDFTLTISSLQPEDFATYYCLQFDHTPFTFGQGTKVEIK

SEQ ID NO: 56 - DNA, 321 bp, Artificial Sequence
  source: /note="Description of Artificial Sequence: Synthetic polynucleotide"
gacatccagatgacccagagcccctccagcctgtccgcctccgtgggcgacagagtgaccatcacctgtcgggcctcccagtccatctcctccaacctgaactggtatcagcagaagcccggcaaggcccctaagctgctgatctacgccgccagcaacctgcagtccggcgtgccctccagattctccggctctggctccggcaccgacttcaccctgaccatctccagcctgcagcccgaggacttcgccacctactactgcctgcagttcgaccacacccctttcaccttcggccagggcaccaaagtggaaatcaag

SEQ ID NO: 57 - protein, 214 aa, Artificial Sequence
  source: /note="Description of Artificial Sequence: Synthetic polypeptide"
DIQMTQSPSSLSASVGDRVTITCRASQSISSNLNWYQQKPGKAPKLLIYAASNLQSGVPSRFSGSGSGTDFTLTISSLQPEDFATYYCLQFDHTPFTFGQGTKVEIKRTVAAPSVFIFPPSDEQLKSGTASVVCLLNNFYPREAKVQWKVDNALQSGNSQESVTEQDSKDSTYSLSSTLTLSKADYEKHKVYACEVTHQGLSSPVTKSFNRGEC

SEQ ID NO: 58 - DNA, 642 bp, Artificial Sequence
  source: /note="Description of Artificial Sequence: Synthetic polynucleotide"
gacatccagatgacccagagcccctccagcctgtccgcctccgtgggcgacagagtgaccatcacctgtcgggcctcccagtccatctcctccaacctgaactggtatcagcagaagcccggcaaggcccctaagctgctgatctacgccgccagcaacctgcagtccggcgtgccctccagattctccggctctggctccggcaccgacttcaccctgaccatctccagcctgcagcccgaggacttcgccacctactactgcctgcagttcgaccacacccctttcaccttcggccagggcaccaaagtggaaatcaagcgtacggtggccgctcccagcgtgttcatcttcccccccagcgacgagcagctgaagagcggcaccgccagcgtggtgtgcctgctgaacaacttctacccccgggaggccaaggtgcagtggaaggtggacaacgccctgcagagcggcaacagccaggagagcgtcaccgagcaggacagcaaggactccacctacagcctgagcagcaccctgaccctgagcaaggccgactacgagaagcataaggtgtacgcctgcgaggtgacccaccagggcctgtccagccccgtgaccaagagcttcaacaggggcgagtgc

SEQ ID NO: 59 - protein, 10 aa, Artificial Sequence
  source: /note="Description of Artificial Sequence: Synthetic peptide"
GFTFSSAAVH

SEQ ID NO: 60 - protein, 19 aa, Artificial Sequence
  source: /note="Description of Artificial Sequence: Synthetic peptide"
RIKSKADGGTTDYAAPVKG

SEQ ID NO: 61 - protein, 18 aa, Artificial Sequence
  source: /note="Description of Artificial Sequence: Synthetic peptide"
DSPSISSYSIPYFSGMDV

SEQ ID NO: 62 - protein, 5 aa, Artificial Sequence
  source: /note="Description of Artificial Sequence: Synthetic peptide"
SAAVH

SEQ ID NO: 63 - protein, 19 aa, Artificial Sequence
  source: /note="Description of Artificial Sequence: Synthetic peptide"
RIKSKADGGTTDYAAPVKG

SEQ ID NO: 64 - protein, 18 aa, Artificial Sequence
  source: /note="Description of Artificial Sequence: Synthetic peptide"
DSPSISSYSIPYFSGMDV

SEQ ID NO: 65 - protein, 7 aa, Artificial Sequence
  source: /note="Description of Artificial Sequence: Synthetic peptide"
GFTFSSA

SEQ ID NO: 66 - protein, 8 aa, Artificial Sequence
  source: /note="Description of Artificial Sequence: Synthetic peptide"
KSKADGGT

SEQ ID NO: 67 - protein, 18 aa, Artificial Sequence
  source: /note="Description of Artificial Sequence: Synthetic peptide"
DSPSISSYSIPYFSGMDV

SEQ ID NO: 68 - protein, 8 aa, Artificial Sequence
  source: /note="Description of Artificial Sequence: Synthetic peptide"
GFTFSSAA

SEQ ID NO: 69 - protein, 10 aa, Artificial Sequence
  source: /note="Description of Artificial Sequence: Synthetic peptide"
IKSKADGGTT

SEQ ID NO: 70 - protein, 20 aa, Artificial Sequence
  source: /note="Description of Artificial Sequence: Synthetic peptide"
ARDSPSISSYSIPYFSGMDV

SEQ ID NO: 71 - protein, 129 aa, Artificial Sequence
  source: /note="Description of Artificial Sequence: Synthetic polypeptide"
QVQLVESGGGLVKPGGSLRLSCAASGFTFSSAAVHWVRQAPGKGLEWVGRIKSKADGGTTDYAAPVKGRFTISRDDSKNTLYLQMNSLKTEDTAVYYCARDSPSISSYSIPYFSGMDVWGQGTLVTVSS

SEQ ID NO: 72 - DNA, 387 bp, Artificial Sequence
  source: /note="Description of Artificial Sequence: Synthetic polynucleotide"
caagtgcagctggtggaatctggcggcggactggtcaagcctggcggtagcctgagactgtcttgcgccgcctccggcttcaccttctcctctgccgctgtgcactgggtccgacaggcccctggcaagggcctggagtgggtcggacggatcaagtccaaggccgacggcggcaccaccgactacgctgcccctgtgaagggccggttcaccatctcccgggacgactccaagaacaccctgtacctgcagatgaactccctgaaaaccgaggacaccgccgtgtactactgcgccagagactccccatctatctccagctactccatcccctacttctccggcatggacgtgtggggccagggcaccctggtcaccgtgtcctct

SEQ ID NO: 73 - protein, 232 aa, Artificial Sequence
  source: /note="Description of Artificial Sequence: Synthetic polypeptide"
QVQLVESGGGLVKPGGSLRLSCAASGFTFSSAAVHWVRQAPGKGLEWVGRIKSKADGGTTDYAAPVKGRFTISRDDSKNTLYLQMNSLKTEDTAVYYCARDSPSISSYSIPYFSGMDVWGQGTLVTVSSASTKGPSVFPLAPSSKSTSGGTAALGCLVKDYFPEPVTVSWNSGALTSGVHTFPAVLQSSGLYSLSSVVTVPSSSLGTQTYICNVNHKPSNTKVDKRVEPKSC

SEQ ID NO: 74 - DNA, 696 bp, Artificial Sequence
  source: /note="Description of Artificial Sequence: Synthetic polynucleotide"
caagtgcagctggtggaatctggcggcggactggtcaagcctggcggtagcctgagactgtcttgcgccgcctccggcttcaccttctcctctgccgctgtgcactgggtccgacaggcccctggcaagggcctggagtgggtcggacggatcaagtccaaggccgacggcggcaccaccgactacgctgcccctgtgaagggccggttcaccatctcccgggacgactccaagaacaccctgtacctgcagatgaactccctgaaaaccgaggacaccgccgtgtactactgcgccagagactccccatctatctccagctactccatcccctacttctccggcatggacgtgtggggccagggcaccctggtcaccgtgtcctctgctagcaccaagggcccctccgtgttccctctggccccttccagcaagtctacctctggcggcaccgctgctctgggctgcctggtgaaggactacttccctgagcctgtgacagtgtcctggaactctggcgccctgacctccggcgtgcacaccttccctgccgtgctgcagtcctccggcctgtactccctgtcctccgtggtgacagtgccttcctccagcctgggcacccagacctatatctgcaacgtgaaccacaagccttccaacaccaaggtggacaagcgggtggagcctaagtcatgc

SEQ ID NO: 75 - protein, 11 aa, Artificial Sequence
  source: /note="Description of Artificial Sequence: Synthetic peptide"
RASQGIRAWLN

SEQ ID NO: 76 - protein, 7 aa, Artificial Sequence
  source: /note="Description of Artificial Sequence: Synthetic peptide"
AASSLQS

SEQ ID NO: 77 - protein, 9 aa, Artificial Sequence
  source: /note="Description of Artificial Sequence: Synthetic peptide"
HQYITHPPT

SEQ ID NO: 78 - protein, 11 aa, Artificial Sequence
  source: /note="Description of Artificial Sequence: Synthetic peptide"
RASQGIRAWLN

SEQ ID NO: 79 - protein, 7 aa, Artificial Sequence
  source: /note="Description of Artificial Sequence: Synthetic peptide"
AASSLQS

SEQ ID NO: 80 - protein, 9 aa, Artificial Sequence
  source: /note="Description of Artificial Sequence: Synthetic peptide"
HQYITHPPT

SEQ ID NO: 81 - protein, 7 aa, Artificial Sequence
  source: /note="Description of Artificial Sequence: Synthetic peptide"
SQGIRAW

SEQ ID NO: 82 - protein, 3 aa, Artificial Sequence
  source: /note="Description of Artificial Sequence: Synthetic peptide"
AAS

SEQ ID NO: 83 - protein, 6 aa, Artificial Sequence
  source: /note="Description of Artificial Sequence: Synthetic peptide"
YITHPP

SEQ ID NO: 84 - protein, 6 aa, Artificial Sequence
  source: /note="Description of Artificial Sequence: Synthetic peptide"
QGIRAW

SEQ ID NO: 85 - protein, 3 aa, Artificial Sequence
  source: /note="Description of Artificial Sequence: Synthetic peptide"
AAS

SEQ ID NO: 86 - protein, 9 aa, Artificial Sequence
  source: /note="Description of Artificial Sequence: Synthetic peptide"
HQYITHPPT

SEQ ID NO: 87 - protein, 107 aa, Artificial Sequence
  source: /note="Description of Artificial Sequence: Synthetic polypeptide"
DIQMTQSPSSLSASVGDRVTITCRASQGIRAWLNWYQQKPGKAPKLLIYAASSLQSGVPSRFSGSGSGTDFTLTISSLQPEDFATYYCHQYITHPPTFGQGTKVEIK

SEQ ID NO: 88 - DNA, 321 bp, Artificial Sequence
  source: /note="Description of Artificial Sequence: Synthetic polynucleotide"
gacatccagatgacccagagcccctccagcctgtccgcctccgtgggcgacagagtgaccatcacctgtcgggcctctcagggcatccgggcctggctgaactggtatcagcagaagcccggcaaggcccctaagctgctgatctacgccgccagctccctgcagtccggcgtgccctccagattctccggctctggctccggcaccgacttcaccctgaccatctccagcctgcagcccgaggacttcgccacctactactgccaccagtacatcacccaccctcccaccttcggccagggcaccaaagtggaaatcaag

SEQ ID NO: 89 - protein, 214 aa, Artificial Sequence
  source: /note="Description of Artificial Sequence: Synthetic polypeptide"
DIQMTQSPSSLSASVGDRVTITCRASQGIRAWLNWYQQKPGKAPKLLIYAASSLQSGVPSRFSGSGSGTDFTLTISSLQPEDFATYYCHQYITHPPTFGQGTKVEIKRTVAAPSVFIFPPSDEQLKSGTASVVCLLNNFYPREAKVQWKVDNALQSGNSQESVTEQDSKDSTYSLSSTLTLSKADYEKHKVYACEVTHQGLSSPVTKSFNRGEC

SEQ ID NO: 90 - DNA, 642 bp, Artificial Sequence
  source: /note="Description of Artificial Sequence: Synthetic polynucleotide"
gacatccagatgacccagagcccctccagcctgtccgcctccgtgggcgacagagtgaccatcacctgtcgggcctctcagggcatccgggcctggctgaactggtatcagcagaagcccggcaaggcccctaagctgctgatctacgccgccagctccctgcagtccggcgtgccctccagattctccggctctggctccggcaccgacttcaccctgaccatctccagcctgcagcccgaggacttcgccacctactactgccaccagtacatcacccaccctcccaccttcggccagggcaccaaagtggaaatcaagcgtacggtggccgctcccagcgtgttcatcttcccccccagcgacgagcagctgaagagcggcaccgccagcgtggtgtgcctgctgaacaacttctacccccgggaggccaaggtgcagtggaaggtggacaacgccctgcagagcggcaacagccaggagagcgtcaccgagcaggacagcaaggactccacctacagcctgagcagcaccctgaccctgagcaaggccgactacgagaagcataaggtgtacgcctgcgaggtgacccaccagggcctgtccagccccgtgaccaagagcttcaacaggggcgagtgc

SEQ ID NO: 91 - protein, 10 aa, Artificial Sequence
  source: /note="Description of Artificial Sequence: Synthetic peptide"
GFTFQSAAVH

SEQ ID NO: 92 - protein, 19 aa, Artificial Sequence
  source: /note="Description of Artificial Sequence: Synthetic peptide"
RIKSKADGGTTDYAAPVKG

SEQ ID NO: 93 - protein, 18 aa, Artificial Sequence
  source: /note="Description of Artificial Sequence: Synthetic peptide"
DSPSISSYSIPYFSGMDV

SEQ ID NO: 94 - protein, 5 aa, Artificial Sequence
  source: /note="Description of Artificial Sequence: Synthetic peptide"
SAAVH

SEQ ID NO: 95 - protein, 19 aa, Artificial Sequence
  source: /note="Description of Artificial Sequence: Synthetic peptide"
RIKSKADGGTTDYAAPVKG

SEQ ID NO: 96 - protein, 18 aa, Artificial Sequence
  source: /note="Description of Artificial Sequence: Synthetic peptide"
DSPSISSYSIPYFSGMDV

SEQ ID NO: 97 - protein, 7 aa, Artificial Sequence
  source: /note="Description of Artificial Sequence: Synthetic peptide"
GFTFQSA

SEQ ID NO: 98 - protein, 8 aa, Artificial Sequence
  source: /note="Description of Artificial Sequence: Synthetic peptide"
KSKADGGT

SEQ ID NO: 99 - protein, 18 aa, Artificial Sequence
  source: /note="Description of Artificial Sequence: Synthetic peptide"
DSPSISSYSIPYFSGMDV

SEQ ID NO: 100 - protein, 8 aa, Artificial Sequence
  source: /note="Description of Artificial Sequence: Synthetic peptide"
GFTFQSAA

SEQ ID NO: 101 - protein, 10 aa, Artificial Sequence
  source: /note="Description of Artificial Sequence: Synthetic peptide"
IKSKADGGTT

SEQ ID NO: 102 - protein, 20 aa, Artificial Sequence
  source: /note="Description of Artificial Sequence: Synthetic peptide"
ARDSPSISSYSIPYFSGMDV

SEQ ID NO: 103 - protein, 129 aa, Artificial Sequence
  source: /note="Description of Artificial Sequence: Synthetic polypeptide"
QVQLVESGGGLVKPGGSLRLSCAASGFTFQSAAVHWVRQAPGKGLEWVGRIKSKADGGTTDYAAPVKGRFTISRDDSKNTLYLQMNSLKTEDTAVYYCARDSPSISSYSIPYFSGMDVWGQGTLVTVSS

SEQ ID NO: 104 - DNA, 387 bp, Artificial Sequence
  source: /note="Description of Artificial Sequence: Synthetic polynucleotide"
caagtgcagctggtggaatctggcggcggactggtcaagcctggcggtagcctgagactgtcttgcgccgcctccggcttcaccttccagtctgccgctgtgcactgggtccgacaggcccctggcaagggcctggagtgggtcggacggatcaagtccaaggccgacggcggcaccaccgactacgctgcccctgtgaagggccggttcaccatctcccgggacgactccaagaacaccctgtacctgcagatgaactccctgaaaaccgaggacaccgccgtgtactactgcgccagagactccccatctatctccagctactccatcccctacttctccggcatggacgtgtggggccagggcaccctggtcaccgtgtcctct

SEQ ID NO: 105 - protein, 232 aa, Artificial Sequence
  source: /note="Description of Artificial Sequence: Synthetic polypeptide"
QVQLVESGGGLVKPGGSLRLSCAASGFTFQSAAVHWVRQAPGKGLEWVGRIKSKADGGTTDYAAPVKGRFTISRDDSKNTLYLQMNSLKTEDTAVYYCARDSPSISSYSIPYFSGMDVWGQGTLVTVSSASTKGPSVFPLAPSSKSTSGGTAALGCLVKDYFPEPVTVSWNSGALTSGVHTFPAVLQSSGLYSLSSVVTVPSSSLGTQTYICNVNHKPSNTKVDKRVEPKSC

SEQ ID NO: 106 - DNA, 696 bp, Artificial Sequence
  source: /note="Description of Artificial Sequence: Synthetic polynucleotide"
caagtgcagctggtggaatctggcggcggactggtcaagcctggcggtagcctgagactgtcttgcgccgcctccggcttcaccttccagtctgccgctgtgcactgggtccgacaggcccctggcaagggcctggagtgggtcggacggatcaagtccaaggccgacggcggcaccaccgactacgctgcccctgtgaagggccggttcaccatctcccgggacgactccaagaacaccctgtacctgcagatgaactccctgaaaaccgaggacaccgccgtgtactactgcgccagagactccccatctatctccagctactccatcccctacttctccggcatggacgtgtggggccagggcaccctggtcaccgtgtcctctgctagcaccaagggcccctccgtgttccctctggccccttccagcaagtctacctctggcggcaccgctgctctgggctgcctggtgaaggactacttccctgagcctgtgacagtgtcctggaactctggcgccctgacctccggcgtgcacaccttccctgccgtgctgcagtcctccggcctgtactccctgtcctccgtggtgacagtgccttcctccagcctgggcacccagacctatatctgcaacgtgaaccacaagccttccaacaccaaggtggacaagcgggtggagcctaagtcatgc

SEQ ID NO: 107 - protein, 11 aa, Artificial Sequence
  source: /note="Description of Artificial Sequence: Synthetic peptide"
RASQGIRAWLN

SEQ ID NO: 108 - protein, 7 aa, Artificial Sequence
  source: /note="Description of Artificial Sequence: Synthetic peptide"
AASSLQS

SEQ ID NO: 109 - protein, 9 aa, Artificial Sequence
  source: /note="Description of Artificial Sequence: Synthetic peptide"
HQYITHPPT

SEQ ID NO: 110 - protein, 11 aa, Artificial Sequence
  source: /note="Description of Artificial Sequence: Synthetic peptide"
RASQGIRAWLN

SEQ ID NO: 111 - protein, 7 aa, Artificial Sequence
  source: /note="Description of Artificial Sequence: Synthetic peptide"
AASSLQS

SEQ ID NO: 112 - protein, 9 aa, Artificial Sequence
  source: /note="Description of Artificial Sequence: Synthetic peptide"
HQYITHPPT

SEQ ID NO: 113 - protein, 7 aa, Artificial Sequence
  source: /note="Description of Artificial Sequence: Synthetic peptide"
SQGIRAW

SEQ ID NO: 114 - protein, 3 aa, Artificial Sequence
  source: /note="Description of Artificial Sequence: Synthetic peptide"
AAS

SEQ ID NO: 115 - protein, 6 aa, Artificial Sequence
  source: /note="Description of Artificial Sequence: Synthetic peptide"
YITHPP

SEQ ID NO: 116 - protein, 6 aa, Artificial Sequence
  source: /note="Description of Artificial Sequence: Synthetic peptide"
QGIRAW

SEQ ID NO: 117 - protein, 3 aa, Artificial Sequence
  source: /note="Description of Artificial Sequence: Synthetic peptide"
AAS

SEQ ID NO: 118 - protein, 9 aa, Artificial Sequence
  source: /note="Description of Artificial Sequence: Synthetic peptide"
HQYITHPPT

SEQ ID NO: 119 - protein, 107 aa, Artificial Sequence; identical to SEQ ID NO: 87
  source: /note="Description of Artificial Sequence: Synthetic polypeptide"

SEQ ID NO: 120 - DNA, 321 bp, Artificial Sequence; identical to SEQ ID NO: 88
  source: /note="Description of Artificial Sequence: Synthetic polynucleotide"

SEQ ID NO: 121 - protein, 214 aa, Artificial Sequence; identical to SEQ ID NO: 89
  source: /note="Description of Artificial Sequence: Synthetic polypeptide"

SEQ ID NO: 122 - DNA, 642 bp, Artificial Sequence; identical to SEQ ID NO: 90
  source: /note="Description of Artificial Sequence: Synthetic polynucleotide"

SEQ ID NO: 123 - protein, 10 aa, Artificial Sequence
  source: /note="Description of Artificial Sequence: Synthetic peptide"
GFTFSSAAVH

SEQ ID NO: 124 - protein, 19 aa, Artificial Sequence
  source: /note="Description of Artificial Sequence: Synthetic peptide"
RIKSKASGGTTDYAAPVKG

SEQ ID NO: 125 - protein, 18 aa, Artificial Sequence
  source: /note="Description of Artificial Sequence: Synthetic peptide"
DSPSISSYSIPYFSGMDV

SEQ ID NO: 126 - protein, 5 aa, Artificial Sequence
  source: /note="Description of Artificial Sequence: Synthetic peptide"
SAAVH

SEQ ID NO: 127 - protein, 19 aa, Artificial Sequence
  source: /note="Description of Artificial Sequence: Synthetic peptide"
RIKSKASGGTTDYAAPVKG

SEQ ID NO: 128 - protein, 18 aa, Artificial Sequence
  source: /note="Description of Artificial Sequence: Synthetic peptide"
DSPSISSYSIPYFSGMDV

SEQ ID NO: 129 - protein, 7 aa, Artificial Sequence
  source: /note="Description of Artificial Sequence: Synthetic peptide"
GFTFSSA

SEQ ID NO: 130 - protein, 8 aa, Artificial Sequence
  source: /note="Description of Artificial Sequence: Synthetic peptide"
KSKASGGT

SEQ ID NO: 131 - protein, 18 aa, Artificial Sequence
  source: /note="Description of Artificial Sequence: Synthetic peptide"
DSPSISSYSIPYFSGMDV

SEQ ID NO: 132 - protein, 8 aa, Artificial Sequence
  source: /note="Description of Artificial Sequence: Synthetic peptide"
GFTFSSAA

SEQ ID NO: 133 - protein, 10 aa, Artificial Sequence
  source: /note="Description of Artificial Sequence: Synthetic peptide"
IKSKASGGTT

SEQ ID NO: 134 - protein, 20 aa, Artificial Sequence
  source: /note="Description of Artificial Sequence: Synthetic peptide"
ARDSPSISSYSIPYFSGMDV

SEQ ID NO: 135 - protein, 129 aa, Artificial Sequence
  source: /note="Description of Artificial Sequence: Synthetic polypeptide"
QVQLVESGGGLVKPGGSLRLSCAASGFTFSSAAVHWVRQAPGKGLEWVGRIKSKASGGTTDYAAPVKGRFTISRDDSKNTLYLQMNSLKTEDTAVYYCARDSPSISSYSIPYFSGMDVWGQGTLVTVSS

SEQ ID NO: 136 - DNA, 387 bp, Artificial Sequence
  source: /note="Description of Artificial Sequence: Synthetic polynucleotide"
caagtgcagctggtggaatctggcggcggactggtcaagcctggcggtagcctgagactgtcttgcgccgcctccggcttcaccttctcctctgccgctgtgcactgggtccgacaggcccctggcaagggcctggagtgggtcggacggatcaagtccaaggcctccggcggcaccaccgactacgctgcccctgtgaagggccggttcaccatctcccgggacgactccaagaacaccctgtacctgcagatgaactccctgaaaaccgaggacaccgccgtgtactactgcgccagagactccccatctatctccagctactccatcccctacttctccggcatggacgtgtggggccagggcaccctggtcaccgtgtcctct

SEQ ID NO: 137 - protein, 232 aa, Artificial Sequence
  source: /note="Description of Artificial Sequence: Synthetic polypeptide"
QVQLVESGGGLVKPGGSLRLSCAASGFTFSSAAVHWVRQAPGKGLEWVGRIKSKASGGTTDYAAPVKGRFTISRDDSKNTLYLQMNSLKTEDTAVYYCARDSPSISSYSIPYFSGMDVWGQGTLVTVSSASTKGPSVFPLAPSSKSTSGGTAALGCLVKDYFPEPVTVSWNSGALTSGVHTFPAVLQSSGLYSLSSVVTVPSSSLGTQTYICNVNHKPSNTKVDKRVEPKSC

SEQ ID NO: 138 - DNA, 696 bp, Artificial Sequence
  source: /note="Description of Artificial Sequence: Synthetic polynucleotide"
caagtgcagctggtggaatctggcggcggactggtcaagcctggcggtagcctgagactgtcttgcgccgcctccggcttcaccttctcctctgccgctgtgcactgggtccgacaggcccctggcaagggcctggagtgggtcggacggatcaagtccaaggcctccggcggcaccaccgactacgctgcccctgtgaagggccggttcaccatctcccgggacgactccaagaacaccctgtacctgcagatgaactccctgaaaaccgaggacaccgccgtgtactactgcgccagagactccccatctatctccagctactccatcccctacttctccggcatggacgtgtggggccagggcaccctggtcaccgtgtcctctgctagcaccaagggcccctccgtgttccctctggccccttccagcaagtctacctctggcggcaccgctgctctgggctgcctggtgaaggactacttccctgagcctgtgacagtgtcctggaactctggcgccctgacctccggcgtgcacaccttccctgccgtgctgcagtcctccggcctgtactccctgtcctccgtggtgacagtgccttcctccagcctgggcacccagacctatatctgcaacgtgaaccacaagccttccaacaccaaggtggacaagcgggtggagcctaagtcatgc

SEQ ID NO: 139 - protein, 11 aa, Artificial Sequence
  source: /note="Description of Artificial Sequence: Synthetic peptide"
RASQGIRAWLN

SEQ ID NO: 140 - protein, 7 aa, Artificial Sequence
  source: /note="Description of Artificial Sequence: Synthetic peptide"
AASSLQS

SEQ ID NO: 141 - protein, 9 aa, Artificial Sequence
  source: /note="Description of Artificial Sequence: Synthetic peptide"
HQYITHPPT

SEQ ID NO: 142 - protein, 11 aa, Artificial Sequence
  source: /note="Description of Artificial Sequence: Synthetic peptide"
RASQGIRAWLN

SEQ ID NO: 143 - protein, 7 aa, Artificial Sequence
  source: /note="Description of Artificial Sequence: Synthetic peptide"
AASSLQS

SEQ ID NO: 144 - protein, 9 aa, Artificial Sequence
  source: /note="Description of Artificial Sequence: Synthetic peptide"
HQYITHPPT

SEQ ID NO: 145 - protein, 7 aa, Artificial Sequence
  source: /note="Description of Artificial Sequence: Synthetic peptide"
SQGIRAW

SEQ ID NO: 146 - protein, 3 aa, Artificial Sequence
  source: /note="Description of Artificial Sequence: Synthetic peptide"
AAS

SEQ ID NO: 147 - protein, 6 aa, Artificial Sequence
  source: /note="Description of Artificial Sequence: Synthetic peptide"
YITHPP

SEQ ID NO: 148 - protein, 6 aa, Artificial Sequence
  source: /note="Description of Artificial Sequence: Synthetic peptide"
QGIRAW

SEQ ID NO: 149 - protein, 3 aa, Artificial Sequence
  source: /note="Description of Artificial Sequence: Synthetic peptide"
AAS

SEQ ID NO: 150 - protein, 9 aa, Artificial Sequence
  source: /note="Description of Artificial Sequence: Synthetic peptide"
HQYITHPPT

SEQ ID NO: 151 - protein, 107 aa, Artificial Sequence; identical to SEQ ID NO: 87
  source: /note="Description of Artificial Sequence: Synthetic polypeptide"

SEQ ID NO: 152 - DNA, 321 bp, Artificial Sequence; identical to SEQ ID NO: 88
  source: /note="Description of Artificial Sequence: Synthetic polynucleotide"

SEQ ID NO: 153 - protein, 214 aa, Artificial Sequence; identical to SEQ ID NO: 89
  source: /note="Description of Artificial Sequence: Synthetic polypeptide"

SEQ ID NO: 154 - DNA, 642 bp, Artificial Sequence; identical to SEQ ID NO: 90
  source: /note="Description of Artificial Sequence: Synthetic polynucleotide"

SEQ ID NO: 155 - protein, 10 aa, Artificial Sequence
  source: /note="Description of Artificial Sequence: Synthetic peptide"
GFTFSSAAVH

SEQ ID NO: 156 - protein, 19 aa, Artificial Sequence
  source: /note="Description of Artificial Sequence: Synthetic peptide"
RIKSKADAGTTDYAAPVKG

SEQ ID NO: 157 - protein, 18 aa, Artificial Sequence
  source: /note="Description of Artificial Sequence: Synthetic peptide"
DSPSISSYSIPYFSGMDV

SEQ ID NO: 158 - protein, 5 aa, Artificial Sequence
  source: /note="Description of Artificial Sequence: Synthetic peptide"
SAAVH

SEQ ID NO: 159 - protein, 19 aa, Artificial Sequence
  source: /note="Description of Artificial Sequence: Synthetic peptide"
RIKSKADAGTTDYAAPVKG

SEQ ID NO: 160 - protein, 18 aa, Artificial Sequence
  source: /note="Description of Artificial Sequence: Synthetic peptide"
DSPSISSYSIPYFSGMDV

SEQ ID NO: 161 - protein, 7 aa, Artificial Sequence
  source: /note="Description of Artificial Sequence: Synthetic peptide"
GFTFSSA

SEQ ID NO: 162 - protein, 8 aa, Artificial Sequence
  source: /note="Description of Artificial Sequence: Synthetic peptide"
KSKADAGT

SEQ ID NO: 163 - protein, 18 aa, Artificial Sequence
  source: /note="Description of Artificial Sequence: Synthetic peptide"
DSPSISSYSIPYFSGMDV

SEQ ID NO: 164 - protein, 8 aa, Artificial Sequence
  source: /note="Description of Artificial Sequence: Synthetic peptide"
GFTFSSAA

SEQ ID NO: 165 - protein, 10 aa, Artificial Sequence
  source: /note="Description of Artificial Sequence: Synthetic peptide"
IKSKADAGTT

SEQ ID NO: 166 - protein, 20 aa, Artificial Sequence
  source: /note="Description of Artificial Sequence: Synthetic peptide"
ARDSPSISSYSIPYFSGMDV

SEQ ID NO: 167 - protein, 129 aa, Artificial Sequence
  source: /note="Description of Artificial Sequence: Synthetic polypeptide"
QVQLVESGGGLVKPGGSLRLSCAASGFTFSSAAVHWVRQAPGKGLEWVGRIKSKADAGTTDYAAPVKGRFTISRDDSKNTLYLQMNSLKTEDTAVYYCARDSPSISSYSIPYFSGMDVWGQGTLVTVSS

SEQ ID NO: 168 - DNA, 387 bp, Artificial Sequence
  source: /note="Description of Artificial Sequence: Synthetic polynucleotide"
caagtgcagctggtggaatctggcggcggactggtcaagcctggcggtagcctgagactgtcttgcgccgcctccggcttcaccttctcctctgccgctgtgcactgggtccgacaggcccctggcaagggcctggagtgggtcggacggatcaagtccaaggccgacgccggcaccaccgactacgctgcccctgtgaagggccggttcaccatctcccgggacgactccaagaacaccctgtacctgcagatgaactccctgaaaaccgaggacaccgccgtgtactactgcgccagagactccccatctatctccagctactccatcccctacttctccggcatggacgtgtggggccagggcaccctggtcaccgtgtcctct

SEQ ID NO: 169 - protein, 232 aa, Artificial Sequence
  source: /note="Description of Artificial Sequence: Synthetic polypeptide"
QVQLVESGGGLVKPGGSLRLSCAASGFTFSSAAVHWVRQAPGKGLEWVGRIKSKADAGTTDYAAPVKGRFTISRDDSKNTLYLQMNSLKTEDTAVYYCARDSPSISSYSIPYFSGMDVWGQGTLVTVSSASTKGPSVFPLAPSSKSTSGGTAALGCLVKDYFPEPVTVSWNSGALTSGVHTFPAVLQSSGLYSLSSVVTVPSSSLGTQTYICNVNHKPSNTKVDKRVEPKSC

SEQ ID NO: 170 - DNA, 696 bp, Artificial Sequence
  source: /note="Description of Artificial Sequence: Synthetic polynucleotide"
caagtgcagctggtggaatctggcggcggactggtcaagcctggcggtagcctgagactgtcttgcgccgcctccggcttcaccttctcctctgccgctgtgcactgggtccgacaggcccctggcaagggcctggagtgggtcggacggatcaagtccaaggccgacgccggcaccaccgactacgctgcccctgtgaagggccggttcaccatctcccgggacgactccaagaacaccctgtacctgcagatgaactccctgaaaaccgaggacaccgccgtgtactactgcgccagagactccccatctatctccagctactccatcccctacttctccggcatggacgtgtggggccagggcaccctggtcaccgtgtcctctgctagcaccaagggcccctccgtgttccctctggccccttccagcaagtctacctctggcggcaccgctgctctgggctgcctggtgaaggactacttccctgagcctgtgacagtgtcctggaactctggcgccctgacctccggcgtgcacaccttccctgccgtgctgcagtcctccggcctgtactccctgtcctccgtggtgacagtgccttcctccagcctgggcacccagacctatatctgcaacgtgaaccacaagccttccaacaccaaggtggacaagcgggtggagcctaagtcatgc

SEQ ID NO: 171 - protein, 11 aa, Artificial Sequence
  source: /note="Description of Artificial Sequence: Synthetic peptide"
RASQGIRAWLN

SEQ ID NO: 172 - protein, 7 aa, Artificial Sequence
  source: /note="Description of Artificial Sequence: Synthetic peptide"
AASSLQS

SEQ ID NO: 173 - protein, 9 aa, Artificial Sequence
  source: /note="Description of Artificial Sequence: Synthetic peptide"
HQYITHPPT

SEQ ID NO: 174 - protein, 11 aa, Artificial Sequence
  source: /note="Description of Artificial Sequence: Synthetic peptide"
RASQGIRAWLN

SEQ ID NO: 175 - protein, 7 aa, Artificial Sequence
  source: /note="Description of Artificial Sequence: Synthetic peptide"
AASSLQS

SEQ ID NO: 176 - protein, 9 aa, Artificial Sequence
  source: /note="Description of Artificial Sequence: Synthetic peptide"
HQYITHPPT

SEQ ID NO: 177 - protein, 7 aa, Artificial Sequence
  source: /note="Description of Artificial Sequence: Synthetic peptide"
SQGIRAW

SEQ ID NO: 178 - protein, 3 aa, Artificial Sequence
  source: /note="Description of Artificial Sequence: Synthetic peptide"
AAS

SEQ ID NO: 179 - protein, 6 aa, Artificial Sequence
  source: /note="Description of Artificial Sequence: Synthetic peptide"
YITHPP

SEQ ID NO: 180 - protein, 6 aa, Artificial Sequence
  source: /note="Description of Artificial Sequence: Synthetic peptide"
QGIRAW

SEQ ID NO: 181 - protein, 3 aa, Artificial Sequence
  source: /note="Description of Artificial Sequence: Synthetic peptide"
AAS

SEQ ID NO: 182 - protein, 9 aa, Artificial Sequence
  source: /note="Description of Artificial Sequence: Synthetic peptide"
HQYITHPPT

SEQ ID NO: 183 - protein, 107 aa, Artificial Sequence; identical to SEQ ID NO: 87
  source: /note="Description of Artificial Sequence: Synthetic polypeptide"

SEQ ID NO: 184 - DNA, 321 bp, Artificial Sequence; identical to SEQ ID NO: 88
  source: /note="Description of Artificial Sequence: Synthetic polynucleotide"

SEQ ID NO: 185 - protein, 214 aa, Artificial Sequence; identical to SEQ ID NO: 89
  source: /note="Description of Artificial Sequence: Synthetic polypeptide"

SEQ ID NO: 186 - DNA, 642 bp, Artificial Sequence; identical to SEQ ID NO: 90
  source: /note="Description of Artificial Sequence: Synthetic polynucleotide"

SEQ ID NO: 187 - protein, 10 aa, Artificial Sequence
  source: /note="Description of Artificial Sequence: Synthetic peptide"
GYSFTNYWIG

SEQ ID NO: 188 - protein, 17 aa, Artificial Sequence
  source: /note="Description of Artificial Sequence: Synthetic peptide"
IIFPGVSYTKYSPSFQG

SEQ ID NO: 189 - protein, 14 aa, Artificial Sequence
  source: /note="Description of Artificial Sequence: Synthetic peptide"
GSDQTLRGSRAMDY

SEQ ID NO: 190 - protein, 5 aa, Artificial Sequence
  source: /note="Description of Artificial Sequence: Synthetic peptide"
NYWIG

SEQ ID NO: 191 - protein, 17 aa, Artificial Sequence
  source: /note="Description of Artificial Sequence: Synthetic peptide"
IIFPGVSYTKYSPSFQG

SEQ ID NO: 192 - protein, 14 aa, Artificial Sequence
  source: /note="Description of Artificial Sequence: Synthetic peptide"
GSDQTLRGSRAMDY

SEQ ID NO: 193 - protein, 7 aa, Artificial Sequence
  source: /note="Description of Artificial Sequence: Synthetic peptide"
GYSFTNY

SEQ ID NO: 194 - protein, 6 aa, Artificial Sequence
  source: /note="Description of Artificial Sequence: Synthetic peptide"
FPGVSY

SEQ ID NO: 195 - protein, 14 aa, Artificial Sequence
  source: /note="Description of Artificial Sequence: Synthetic peptide"
GSDQTLRGSRAMDY

SEQ ID NO: 196 - protein, 8 aa, Artificial Sequence
  source: /note="Description of Artificial Sequence: Synthetic peptide"
GYSFTNYW

SEQ ID NO: 197 - protein, 8 aa, Artificial Sequence
  source: /note="Description of Artificial Sequence: Synthetic peptide"
IFPGVSYT

SEQ ID NO: 198 - protein, 16 aa, Artificial Sequence
  source: /note="Description of Artificial Sequence: Synthetic peptide"
ARGSDQTLRGSRAMDY

SEQ ID NO: 199 - protein, 123 aa, Artificial Sequence
  source: /note="Description of Artificial Sequence: Synthetic polypeptide"
QVQLVQSGAEVKKPGESLKISCKGSGYSFTNYWIGWVRQMPGKGLEWMGIIFPGVSYTKYSPSFQGQVTISADKSISTAYLQWSSLKASDTAMYYCARGSDQTLRGSRAMDYWGQGTLVTVSS

SEQ ID NO: 200 - DNA, 369 bp, Artificial Sequence
  source: /note="Description of Artificial Sequence: Synthetic polynucleotide"
caagtgcagctggtgcagtctggcgctgaagtgaagaagcccggcgagtccctgaagatctcctgcaagggctccggctactccttcaccaactactggatcggctgggtccgacagatgcccggcaagggcctggagtggatgggcatcatcttccccggcgtgtcctacaccaagtacagccccagcttccagggccaagtcacaatctccgccgacaagtccatctccaccgcctacctgcagtggtcctccctgaaggcctccgacaccgccatgtactactgcgccagaggctccgaccagaccctgcggggctccagagccatggattactggggccagggcaccctggtcaccgtgtcctct

SEQ ID NO: 201 - protein, 226 aa, Artificial Sequence
  source: /note="Description of Artificial Sequence: Synthetic polypeptide"
QVQLVQSGAEVKKPGESLKISCKGSGYSFTNYWIGWVRQMPGKGLEWMGIIFPGVSYTKYSPSFQGQVTISADKSISTAYLQWSSLKASDTAMYYCARGSDQTLRGSRAMDYWGQGTLVTVSSASTKGPSVFPLAPSSKSTSGGTAALGCLVKDYFPEPVTVSWNSGALTSGVHTFPAVLQSSGLYSLSSVVTVPSSSLGTQTYICNVNHKPSNTKVDKRVEPKSC

SEQ ID NO: 202 - DNA, 678 bp, Artificial Sequence
  source: /note="Description of Artificial Sequence: Synthetic polynucleotide"
caagtgcagctggtgcagtctggcgctgaagtgaagaagcccggcgagtccctgaagatctcctgcaagggctccggctactccttcaccaactactggatcggctgggtccgacagatgcccggcaagggcctggagtggatgggcatcatcttccccggcgtgtcctacaccaagtacagccccagcttccagggccaagtcacaatctccgccgacaagtccatctccaccgcctacctgcagtggtcctccctgaaggcctccgacaccgccatgtactactgcgccagaggctccgaccagaccctgcggggctccagagccatggattactggggccagggcaccctggtcaccgtgtcctctgctagcaccaagggcccctccgtgttccctctggccccttccagcaagtctacctctggcggcaccgctgctctgggctgcctggtgaaggactacttccctgagcctgtgacagtgtcctggaactctggcgccctgacctccggcgtgcacaccttccctgccgtgctgcagtcctccggcctgtactccctgtcctccgtggtgacagtgccttcctccagcctgggcacccagacctatatctgcaacgtgaaccacaagccttccaacaccaaggtggacaagcgggtggagcctaagtcatgc

SEQ ID NO: 203 - protein, 14 aa, Artificial Sequence
  source: /note="Description of Artificial Sequence: Synthetic peptide"
TGTSSDVGISNYVS

SEQ ID NO: 204 - protein, 7 aa, Artificial Sequence
  source: /note="Description of Artificial Sequence: Synthetic peptide"
EVSNRPS

SEQ ID NO: 205 - protein, 9 aa, Artificial Sequence
  source: /note="Description of Artificial Sequence: Synthetic peptide"
QSYTSLNYV

SEQ ID NO: 206 - protein, 14 aa, Artificial Sequence
  source: /note="Description of Artificial Sequence: Synthetic peptide"
TGTSSDVGISNYVS

SEQ ID NO: 207 - protein, 7 aa, Artificial Sequence
  source: /note="Description of Artificial Sequence: Synthetic peptide"
EVSNRPS

SEQ ID NO: 208 - protein, 9 aa, Artificial Sequence
  source: /note="Description of Artificial Sequence: Synthetic peptide"
QSYTSLNYV

SEQ ID NO: 209 - protein, 10 aa, Artificial Sequence
  source: /note="Description of Artificial Sequence: Synthetic peptide"
TSSDVGISNY

SEQ ID NO: 210 - protein, 3 aa, Artificial Sequence
  source: /note="Description of Artificial Sequence: Synthetic peptide"
EVS

SEQ ID NO: 211 - protein, 6 aa, Artificial Sequence
  source: /note="Description of Artificial Sequence: Synthetic peptide"
YTSLNY

SEQ ID NO: 212 - protein, 9 aa, Artificial Sequence
  source: /note="Description of Artificial Sequence: Synthetic peptide"
SSDVGISNY

SEQ ID NO: 213 - protein, 3 aa, Artificial Sequence
  source: /note="Description of Artificial Sequence: Synthetic peptide"
EVS

SEQ ID NO: 214 - protein, 9 aa, Artificial Sequence
  source: /note="Description of Artificial Sequence: Synthetic peptide"
QSYTSLNYV

SEQ ID NO: 215 - protein, 109 aa, Artificial Sequence
  source: /note="Description of Artificial Sequence: Synthetic polypeptide"
QSALTQPASVSGSPGQSITISCTGTSSDVGISNYVSWYQQHPGKAPKLMIYEVSNRPSGVSNRFSGSKSGNTASLTISGLQAEDEADYYCQSYTSLNYVFGGGTKLTVL

SEQ ID NO: 216 - DNA, 327 bp, Artificial Sequence
  source: /note="Description of Artificial Sequence: Synthetic polynucleotide"
cagtccgccctgacccagcctgcctccgtgtctggctcccctggccagtccatcaccatcagctgcaccggcacctccagcgacgtgggcatctccaactacgtgtcctggtatcagcagcaccccggcaaggcccctaagctgatgatctacgaagtgtccaaccggccctccggcgtgtccaacagattctccggctccaagtccggcaacaccgcctccctgaccatcagcggcctgcaggctgaggacgaggccgactactactgccagtcctacacctccctgaactacgtgttcggcggaggcaccaagctgaccgtgctg

SEQ ID NO: 217 - protein, 215 aa, Artificial Sequence
  source: /note="Description of Artificial Sequence: Synthetic polypeptide"
QSALTQPASVSGSPGQSITISCTGTSSDVGISNYVSWYQQHPGKAPKLMIYEVSNRPSGVSNRFSGSKSGNTASLTISGLQAEDEADYYCQSYTSLNYVFGGGTKLTVLGQPKAAPSVTLFPPSSEELQANKATLVCLISDFYPGAVTVAWKADSSPVKAGVETTTPSKQSNNKYAASSYLSLTPEQWKSHRSYSCQVTHEGSTVEKTVAPTECS

SEQ ID NO: 218 - DNA, 645 bp, Artificial Sequence
  source: /note="Description of Artificial Sequence: Synthetic polynucleotide"
cagtccgccctgacccagcctgcctccgtgtctggctcccctggccagtccatcaccatcagctgcaccggcacctccagcgacgtgggcatctccaactacgtgtcctggtatcagcagcaccccggcaaggcccctaagctgatgatctacgaagtgtccaaccggccctccggcgtgtccaacagattctccggctccaagtccggcaacaccgcctccctgaccatcagcggcctgcaggctgaggacgaggccgactactactgccagtcctacacctccctgaactacgtgttcggcggaggcaccaagctgaccgtgctgggccagcctaaggctgcccccagcgtgaccctgttcccccccagcagcgaggagctgcaggccaacaaggccaccctggtgtgcctgatcagcgacttctacccaggcgccgtgaccgtggcctggaaggccgacagcagccccgtgaaggccggcgtggagaccaccacccccagcaagcagagcaacaacaagtacgccgccagcagctacctgagcctgacccccgagcagtggaagagccacaggtcctacagctgccaggtgacccacgagggcagcaccgtggaaaagaccgtggccccaaccgagtgcagc

SEQ ID NO: 219 - protein, 10 aa, Artificial Sequence
  source: /note="Description of Artificial Sequence: Synthetic peptide"
GFTFSSNAMH

SEQ ID NO: 220 - protein, 19 aa, Artificial Sequence
  source: /note="Description of Artificial Sequence: Synthetic peptide"
RIKSKTDGGTTDYAAPVKG

SEQ ID NO: 221 - protein, 9 aa, Artificial Sequence
  source: /note="Description of Artificial Sequence: Synthetic peptide"
DHYYYPFAY

SEQ ID NO: 222 - protein, 5 aa, Artificial Sequence
  source: /note="Description of Artificial Sequence: Synthetic peptide"
SNAMH

SEQ ID NO: 223 - protein, 19 aa, Artificial Sequence
  source: /note="Description of Artificial Sequence: Synthetic peptide"
RIKSKTDGGTTDYAAPVKG

SEQ ID NO: 224 - protein, 9 aa, Artificial Sequence
  source: /note="Description of Artificial Sequence: Synthetic peptide"
DHYYYPFAY

SEQ ID NO: 225 - protein, 7 aa, Artificial Sequence
  source: /note="Description of Artificial Sequence: Synthetic peptide"
GFTFSSN

SEQ ID NO: 226 - protein, 8 aa, Artificial Sequence
  source: /note="Description of Artificial Sequence: Synthetic peptide"
KSKTDGGT

SEQ ID NO: 227 - protein, 9 aa, Artificial Sequence
  source: /note="Description of Artificial Sequence: Synthetic peptide"
DHYYYPFAY

SEQ ID NO: 228 - protein, 8 aa, Artificial Sequence
  source: /note="Description of Artificial Sequence: Synthetic peptide"
GFTFSSNA

SEQ ID NO: 229 - protein, 10 aa, Artificial Sequence
  source: /note="Description of Artificial Sequence: Synthetic peptide"
IKSKTDGGTT

SEQ ID NO: 230 - protein, 11 aa, Artificial Sequence
  source: /note="Description of Artificial Sequence: Synthetic peptide"
ARDHYYYPFAY

SEQ ID NO: 231 - protein, 120 aa, Artificial Sequence
  source: /note="Description of Artificial Sequence: Synthetic polypeptide"
QVQLVESGGGLVKPGGSLRLSCAASGFTFSSNAMHWVRQAPGKGLEWVGRIKSKTDGGTTDYAAPVKGRFTISRDDSKNTLYLQMNSLKTEDTAVYYCARDHYYYPFAYWGQGTLVTVSS

SEQ ID NO: 232 - DNA, 360 bp, Artificial Sequence
  source: /note="Description of Artificial Sequence: Synthetic polynucleotide"
caagtgcagctggtggaatctggcggcggactggtcaagcctggcggtagcctgagactgtcttgcgccgcctccggcttcaccttctcctccaacgccatgcactgggtccgacaggcccctggcaagggcctggagtgggtcggacggatcaagtccaagaccgacggcggcaccaccgactacgctgcccctgtgaagggccggttcaccatctcccgggacgactccaagaacaccctgtacctgcagatgaactccctgaaaaccgaggacaccgccgtgtactactgcgccagggaccactactactaccccttcgcctactggggccagggcaccctggtcaccgtgtcctct

SEQ ID NO: 233 - protein, 223 aa, Artificial Sequence
  source: /note="Description of Artificial Sequence: Synthetic polypeptide"
QVQLVESGGGLVKPGGSLRLSCAASGFTFSSNAMHWVRQAPGKGLEWVGRIKSKTDGGTTDYAAPVKGRFTISRDDSKNTLYLQMNSLKTEDTAVYYCARDHYYYPFAYWGQGTLVTVSSASTKGPSVFPLAPSSKSTSGGTAALGCLVKDYFPEPVTVSWNSGALTSGVHTFPAVLQSSGLYSLSSVVTVPSSSLGTQTYICNVNHKPSNTKVDKRVEPKSC

SEQ ID NO: 234 - DNA, 669 bp, Artificial Sequence
  source: /note="Description of Artificial Sequence: Synthetic polynucleotide"
caagtgcagctggtggaatctggcggcggactggtcaagcctggcggtagcctgagactgtcttgcgccgcctccggcttcaccttctcctccaacgccatgcactgggtccgacaggcccctggcaagggcctggagtgggtcggacggatcaagtccaagaccgacggcggcaccaccgactacgctgcccctgtgaagggccggttcaccatctcccgggacgactccaagaacaccctgtacctgcagatgaactccctgaaaaccgaggacaccgccgtgtactactgcgccagggaccactactactaccccttcgcctactggggccagggcaccctggtcaccgtgtcctctgctagcaccaagggcccctccgtgttccctctggccccttccagcaagtctacctctggcggcaccgctgctctgggctgcctggtgaaggactacttccctgagcctgtgacagtgtcctggaactctggcgccctgacctccggcgtgcacaccttccctgccgtgctgcagtcctccggcctgtactccctgtcctccgtggtgacagtgccttcctccagcctgggcacccagacctatatctgcaacgtgaaccacaagccttccaacaccaaggtggacaagcgggtggagcctaagtcatgc

SEQ ID NO: 235 - protein, 11 aa, Artificial Sequence
  source: /note="Description of Artificial Sequence: Synthetic peptide"
RASQSIRYNLA

SEQ ID NO: 236 - protein, 7 aa, Artificial Sequence
  source: /note="Description of Artificial Sequence: Synthetic peptide"
AASSLQS

SEQ ID NO: 237 - protein, 9 aa, Artificial Sequence
  source: /note="Description of Artificial Sequence: Synthetic peptide"
HQYIAKPIT

SEQ ID NO: 238 - protein, 11 aa, Artificial Sequence
  source: /note="Description of Artificial Sequence: Synthetic peptide"
RASQSIRYNLA

SEQ ID NO: 239 - protein, 7 aa, Artificial Sequence
  source: /note="Description of Artificial Sequence: Synthetic peptide"
AASSLQS

SEQ ID NO: 240 - protein, 9 aa, Artificial Sequence
  source: /note="Description of Artificial Sequence: Synthetic peptide"
HQYIAKPIT

SEQ ID NO: 241 - protein, 7 aa, Artificial Sequence
  source: /note="Description of Artificial Sequence: Synthetic peptide"
SQSIRYN

SEQ ID NO: 242 - protein, 3 aa, Artificial Sequence
  source: /note="Description of Artificial Sequence: Synthetic peptide"
AAS

SEQ ID NO: 243 - protein, 6 aa, Artificial Sequence
  source: /note="Description of Artificial Sequence: Synthetic peptide"
YIAKPI

SEQ ID NO: 244 - protein, 6 aa, Artificial Sequence
  source: /note="Description of Artificial Sequence: Synthetic peptide"
QSIRYN

SEQ ID NO: 245 - protein, 3 aa, Artificial Sequence
  source: /note="Description of Artificial Sequence: Synthetic peptide"
AAS

SEQ ID NO: 246 - protein, 9 aa, Artificial Sequence
  source: /note="Description of Artificial Sequence: Synthetic peptide"
HQYIAKPIT

SEQ ID NO: 247 - protein, 107 aa, Artificial Sequence
  source: /note="Description of Artificial Sequence: Synthetic polypeptide"
DIQMTQSPSSLSASVGDRVTITCRASQSIRYNLAWYQQKPGKAPKLLIYAASSLQSGVPSRFSGSGSGTDFTLTISSLQPEDFATYYCHQYIAKPITFGQGTKVEIK

SEQ ID NO: 248 - DNA, 321 bp, Artificial Sequence
  source: /note="Description of Artificial Sequence: Synthetic polynucleotide"
gacatccagatgacccagagcccctccagcctgtccgcctccgtgggcgacagagtgaccatcacctgtcgggcctcccagtccatccggtacaacctggcctggtatcagcagaagcccggcaaggcccctaagctgctgatctacgccgccagctccctgcagtccggcgtgccctccagattctccggctctggctccggcaccgacttcaccctgaccatctccagcctgcagcccgaggacttcgccacctactactgccaccagtatatcgccaagcccatcaccttcggccagggcaccaaagtggaaatcaag

SEQ ID NO: 249 - protein, 214 aa, Artificial Sequence
  source: /note="Description of Artificial Sequence: Synthetic polypeptide"
DIQMTQSPSSLSASVGDRVTITCRASQSIRYNLAWYQQKPGKAPKLLIYAASSLQSGVPSRFSGSGSGTDFTLTISSLQPEDFATYYCHQYIAKPITFGQGTKVEIKRTVAAPSVFIFPPSDEQLKSGTASVVCLLNNFYPREAKVQWKVDNALQSGNSQESVTEQDSKDSTYSLSSTLTLSKADYEKHKVYACEVTHQGLSSPVTKSFNRGEC

SEQ ID NO: 250 - DNA, 642 bp, Artificial Sequence
  source: /note="Description of Artificial Sequence: Synthetic polynucleotide"
gacatccagatgacccagagcccctccagcctgtccgcctccgtgggcgacagagtgaccatcacctgtcgggcctcccagtccatccggtacaacctggcctggtatcagcagaagcccggcaaggcccctaagctgctgatctacgccgccagctccctgcagtccggcgtgccctccagattctccggctctggctccggcaccgacttcaccctgaccatctccagcctgcagcccgaggacttcgccacctactactgccaccagtatatcgccaagcccatcaccttcggccagggcaccaaagtggaaatcaagcgtacggtggccgctcccagcgtgttcatcttcccccccagcgacgagcagctgaagagcggcaccgccagcgtggtgtgcctgctgaacaacttctacccccgggaggccaaggtgcagtggaaggtggacaacgccctgcagagcggcaacagccaggagagcgtcaccgagcaggacagcaaggactccacctacagcctgagcagcaccctgaccctgagcaaggccgactacgagaagcataaggtgtacgcctgcgaggtgacccaccagggcctgtccagccccgtgaccaagagcttcaacaggggcgagtgc

SEQ ID NO: 251 - protein, 10 aa, Artificial Sequence
  source: /note="Description of Artificial Sequence: Synthetic peptide"
GFTFSSNAMH

SEQ ID NO: 252 - protein, 19 aa, Artificial Sequence
  source: /note="Description of Artificial Sequence: Synthetic peptide"
RIKSKTSGGTTDYAAPVKG

SEQ ID NO: 253 - protein, 9 aa, Artificial Sequence
  source: /note="Description of Artificial Sequence: Synthetic peptide"
DHYYYPFAY

SEQ ID NO: 254 - protein, 5 aa, Artificial Sequence
  source: /note="Description of Artificial Sequence: Synthetic peptide"
SNAMH

SEQ ID NO: 255 - protein, 19 aa, Artificial Sequence
  source: /note="Description of Artificial Sequence: Synthetic peptide"
RIKSKTSGGTTDYAAPVKG

SEQ ID NO: 256 - protein, 9 aa, Artificial Sequence
  source: /note="Description of Artificial Sequence: Synthetic peptide"
DHYYYPFAY

SEQ ID NO: 257 - protein, 7 aa, Artificial Sequence
  source: /note="Description of Artificial Sequence: Synthetic peptide"
GFTFSSN

SEQ ID NO: 258 - protein, 8 aa, Artificial Sequence
  source: /note="Description of Artificial Sequence: Synthetic peptide"
KSKTSGGT

SEQ ID NO: 259 - protein, 9 aa, Artificial Sequence
  source: /note="Description of Artificial Sequence: Synthetic peptide"
DHYYYPFAY

SEQ ID NO: 260 - protein, 8 aa, Artificial Sequence
  source: /note="Description of Artificial Sequence: Synthetic peptide"
GFTFSSNA

SEQ ID NO: 261 - protein, 10 aa, Artificial Sequence
  source: /note="Description of Artificial Sequence: Synthetic peptide"
IKSKTSGGTT

SEQ ID NO: 262 - protein, 11 aa, Artificial Sequence
  source: /note="Description of Artificial Sequence: Synthetic peptide"
ARDHYYYPFAY

SEQ ID NO: 263 - protein, 120 aa, Artificial Sequence
  source: /note="Description of Artificial Sequence: Synthetic polypeptide"
QVQLVESGGGLVKPGGSLRLSCAASGFTFSSNAMHWVRQAPGKGLEWVGRIKSKTSGGTTDYAAPVKGRFTISRDDSKNTLYLQMNSLKTEDTAVYYCARDHYYYPFAYWGQGTLVTVSS

SEQ ID NO: 264 - DNA, 360 bp, Artificial Sequence
  source: /note="Description of Artificial Sequence: Synthetic polynucleotide"
caagtgcagctggtggaatctggcggcggactggtcaagcctggcggtagcctgagactgtcttgcgccgcctccggcttcaccttctcctccaacgccatgcactgggtccgacaggcccctggcaagggcctggagtgggtcggacggatcaagtccaagacctccggcggcaccaccgactacgctgcccctgtgaagggccggttcaccatctcccgggacgactccaagaacaccctgtacctgcagatgaactccctgaaaaccgaggacaccgccgtgtactactgcgccagggaccactactactaccccttcgcctactggggccagggcaccctggtcaccgtgtcctct

SEQ ID NO: 265 - protein, 223 aa, Artificial Sequence
  source: /note="Description of Artificial Sequence: Synthetic polypeptide"
QVQLVESGGGLVKPGGSLRLSCAASGFTFSSNAMHWVRQAPGKGLEWVGRIKSKTSGGTTDYAAPVKGRFTISRDDSKNTLYLQMNSLKTEDTAVYYCARDHYYYPFAYWGQGTLVTVSSASTKGPSVFPLAPSSKSTSGGTAALGCLVKDYFPEPVTVSWNSGALTSGVHTFPAVLQSSGLYSLSSVVTVPSSSLGTQTYICNVNHKPSNTKVDKRVEPKSC

SEQ ID NO: 266 - DNA, 669 bp, Artificial Sequence
  source: /note="Description of Artificial Sequence: Synthetic polynucleotide"
caagtgcagctggtggaatctggcggcggactggtcaagcctggcggtagcctgagactgtcttgcgccgcctccggcttcaccttctcctccaacgccatgcactgggtccgacaggcccctggcaagggcctggagtgggtcggacggatcaagtccaagacctccggcggcaccaccgactacgctgcccctgtgaagggccggttcaccatctcccgggacgactccaagaacaccctgtacctgcagatgaactccctgaaaaccgaggacaccgccgtgtactactgcgccagggaccactactactaccccttcgcctactggggccagggcaccctggtcaccgtgtcctctgctagcaccaagggcccctccgtgttccctctggccccttccagcaagtctacctctggcggcaccgctgctctgggctgcctggtgaaggactacttccctgagcctgtgacagtgtcctggaactctggcgccctgacctccggcgtgcacaccttccctgccgtgctgcagtcctccggcctgtactccctgtcctccgtggtgacagtgccttcctccagcctgggcacccagacctatatctgcaacgtgaaccacaagccttccaacaccaaggtggacaagcgggtggagcctaagtcatgc

SEQ ID NO: 267 - protein, 11 aa, Artificial Sequence
  source: /note="Description of Artificial Sequence: Synthetic peptide"
RASQSIRYNLA

SEQ ID NO: 268 - protein, 7 aa, Artificial Sequence
  source: /note="Description of Artificial Sequence: Synthetic peptide"
AASSLQS

SEQ ID NO: 269 - protein, 9 aa, Artificial Sequence
  source: /note="Description of Artificial Sequence: Synthetic peptide"
HQYIAKPIT

SEQ ID NO: 270 - protein, 11 aa, Artificial Sequence
  source: /note="Description of Artificial Sequence: Synthetic peptide"
RASQSIRYNLA

SEQ ID NO: 271 - protein, 7 aa, Artificial Sequence
  source: /note="Description of Artificial Sequence: Synthetic peptide"
AASSLQS

SEQ ID NO: 272 - protein, 9 aa, Artificial Sequence
  source: /note="Description of Artificial Sequence: Synthetic peptide"
HQYIAKPIT

SEQ ID NO: 273 - protein, 7 aa, Artificial Sequence
  source: /note="Description of Artificial Sequence: Synthetic peptide"
SQSIRYN

SEQ ID NO: 274 - protein, 3 aa, Artificial Sequence
  source: /note="Description of Artificial Sequence: Synthetic peptide"
AAS

SEQ ID NO: 275 - protein, 6 aa, Artificial Sequence
  source: /note="Description of Artificial Sequence: Synthetic peptide"
YIAKPI

SEQ ID NO: 276 - protein, 6 aa, Artificial Sequence
  source: /note="Description of Artificial Sequence: Synthetic peptide"
QSIRYN

SEQ ID NO: 277 - protein, 3 aa, Artificial Sequence
  source: /note="Description of Artificial Sequence: Synthetic peptide"
AAS

SEQ ID NO: 278 - protein, 9 aa, Artificial Sequence
  source: /note="Description of Artificial Sequence: Synthetic peptide"
HQYIAKPIT

SEQ ID NO: 279 - protein, 107 aa, Artificial Sequence; identical to SEQ ID NO: 247
  source: /note="Description of Artificial Sequence: Synthetic polypeptide"

SEQ ID NO: 280 - DNA, 321 bp, Artificial Sequence; identical to SEQ ID NO: 248
  source: /note="Description of Artificial Sequence: Synthetic polynucleotide"

SEQ ID NO: 281 - protein, 214 aa, Artificial Sequence; identical to SEQ ID NO: 249
  source: /note="Description of Artificial Sequence: Synthetic polypeptide"

SEQ ID NO: 282 - DNA, 642 bp, Artificial Sequence; identical to SEQ ID NO: 250
  source: /note="Description of Artificial Sequence: Synthetic polynucleotide"

SEQ ID NO: 283 - protein, 10 aa, Artificial Sequence
  source: /note="Description of Artificial Sequence: Synthetic peptide"
GYTFTNYYVH

SEQ ID NO: 284 - protein, 17 aa, Artificial Sequence
  source: /note="Description of Artificial Sequence: Synthetic peptide"
WINPYNGNTNYAQKFQG

SEQ ID NO: 285 - protein, 13 aa, Artificial Sequence
  source: /note="Description of Artificial Sequence: Synthetic peptide"
GASSIRMSYYLDV

SEQ ID NO: 286 - protein, 5 aa, Artificial Sequence
  source: /note="Description of Artificial Sequence: Synthetic peptide"
NYYVH

SEQ ID NO: 287 - protein, 17 aa, Artificial Sequence
  source: /note="Description of Artificial Sequence: Synthetic peptide"
WINPYNGNTNYAQKFQG

SEQ ID NO: 288 - protein, 13 aa, Artificial Sequence
  source: /note="Description of Artificial Sequence: Synthetic peptide"
GASSIRMSYYLDV

SEQ ID NO: 289 - protein, 7 aa, Artificial Sequence
  source: /note="Description of Artificial Sequence: Synthetic peptide"
GYTFTNY

SEQ ID NO: 290 - protein, 6 aa, Artificial Sequence
  source: /note="Description of Artificial Sequence: Synthetic peptide"
NPYNGN

SEQ ID NO: 291 - protein, 13 aa, Artificial Sequence
  source: /note="Description of Artificial Sequence: Synthetic peptide"
GASSIRMSYYLDV

SEQ ID NO: 292 - protein, 8 aa, Artificial Sequence
  source: /note="Description of Artificial Sequence: Synthetic peptide"
GYTFTNYY

SEQ ID NO: 293 - protein, 8 aa, Artificial Sequence
  source: /note="Description of Artificial Sequence: Synthetic peptide"
INPYNGNT

SEQ ID NO: 294 - protein, 15 aa, Artificial Sequence
  source: /note="Description of Artificial Sequence: Synthetic peptide"
ARGASSIRMSYYLDV

SEQ ID NO: 295 - protein, 122 aa, Artificial Sequence
  source: /note="Description of Artificial Sequence: Synthetic polypeptide"
QVQLVQSGAEVKKPGASVKVSCKASGYTFTNYYVHWVRQAPGQGLEWMGWINPYNGNTNYAQKFQGRVTMTRDTSISTAYMELSRLRSEDTAVYYCARGASSIRMSYYLDVWGQGTLVTVSS

SEQ ID NO: 296 - DNA, 366 bp, Artificial Sequence
  source: /note="Description of Artificial Sequence: Synthetic polynucleotide"
caagtgcagctggtgcagtctggcgctgaagtgaagaaacctggcgcctccgtgaaagtgtcctgcaaggcctccggctacaccttcaccaactactacgtgcactgggtccgacaggccccaggccagggcctggagtggatgggctggatcaacccctacaacggcaacaccaactacgcccagaaattccagggcagagtgaccatgacccgggacacctccatctccaccgcctacatggaactgtcccggctgcggagcgaggacaccgccgtgtactactgtgccagaggcgcctcctccatccggatgtcctactacctggacgtgtggggccagggcaccctggtcaccgtgtcctct

SEQ ID NO: 297 - protein, 225 aa, Artificial Sequence
  source: /note="Description of Artificial Sequence: Synthetic polypeptide"
QVQLVQSGAEVKKPGASVKVSCKASGYTFTNYYVHWVRQAPGQGLEWMGWINPYNGNTNYAQKFQGRVTMTRDTSISTAYMELSRLRSEDTAVYYCARGASSIRMSYYLDVWGQGTLVTVSSASTKGPSVFPLAPSSKSTSGGTAALGCLVKDYFPEPVTVSWNSGALTSGVHTFPAVLQSSGLYSLSSVVTVPSSSLGTQTYICNVNHKPSNTKVDKRVEPKSC

SEQ ID NO: 298 - DNA, 675 bp, Artificial Sequence
  source: /note="Description of Artificial Sequence: Synthetic polynucleotide"
caagtgcagctggtgcagtctggcgctgaagtgaagaaacctggcgcctccgtgaaagtgtcctgcaaggcctccggctacaccttcaccaactactacgtgcactgggtccgacaggccccaggccagggcctggagtggatgggctggatcaacccctacaacggcaacaccaactacgcccagaaattccagggcagagtgaccatgacccgggacacctccatctccaccgcctacatggaactgtcccggctgcggagcgaggacaccgccgtgtactactgtgccagaggcgcctcctccatccggatgtcctactacctggacgtgtggggccagggcaccctggtcaccgtgtcctctgctagcaccaagggcccctccgtgttccctctggccccttccagcaagtctacctctggcggcaccgctgctctgggctgcctggtgaaggactacttccctgagcctgtgacagtgtcctggaactctggcgccctgacctccggcgtgcacaccttccctgccgtgctgcagtcctccggcctgtactccctgtcctccgtggtgacagtgccttcctccagcctgggcacccagacctatatctgcaacgtgaaccacaagccttccaacaccaaggtggacaagcgggtggagcctaagtcatgc

SEQ ID NO: 299 - protein, 11 aa, Artificial Sequence
  source: /note="Description of Artificial Sequence: Synthetic peptide"
RASQSISNYLN

SEQ ID NO: 300 - protein, 7 aa, Artificial Sequence
  source: /note="Description of Artificial Sequence: Synthetic peptide"
AASNLQS

SEQ ID NO: 301 - protein, 9 aa, Artificial Sequence
  source: /note="Description of Artificial Sequence: Synthetic peptide"
FQYTHSPAT

SEQ ID NO: 302 - protein, 11 aa, Artificial Sequence
  source: /note="Description of Artificial Sequence: Synthetic peptide"
RASQSISNYLN

SEQ ID NO: 303 - protein, 7 aa, Artificial Sequence
  source: /note="Description of Artificial Sequence: Synthetic peptide"
AASNLQS

SEQ ID NO: 304 - protein, 9 aa, Artificial Sequence
  source: /note="Description of Artificial Sequence: Synthetic peptide"
FQYTHSPAT

SEQ ID NO: 305 - protein, 7 aa, Artificial Sequence
  source: /note="Description of Artificial Sequence: Synthetic peptide"
SQSISNY

SEQ ID NO: 306 - protein, 3 aa, Artificial Sequence
  source: /note="Description of Artificial Sequence: Synthetic peptide"
AAS

SEQ ID NO: 307 - protein, 6 aa, Artificial Sequence
  source: /note="Description of Artificial Sequence: Synthetic peptide"
YTHSPA

SEQ ID NO: 308 - protein, 6 aa, Artificial Sequence
  source: /note="Description of Artificial Sequence: Synthetic peptide"
QSISNY

SEQ ID NO: 309 - protein, 3 aa, Artificial Sequence
  source: /note="Description of Artificial Sequence: Synthetic peptide"
AAS

SEQ ID NO: 310 - protein, 9 aa, Artificial Sequence
  source: /note="Description of Artificial Sequence: Synthetic peptide"
FQYTHSPAT

SEQ ID NO: 311 - protein, 107 aa, Artificial Sequence
  source: /note="Description of Artificial Sequence: Synthetic polypeptide"
DIQMTQSPSSLSASVGDRVTITCRASQSISNYLNWYQQKPGKAPKLLIYAASNLQSGVPSRFSGSGSGTDFTLTISSLQPEDFATYYCFQYTHSPATFGQGTKVEIK

SEQ ID NO: 312 - DNA, 321 bp, Artificial Sequence
  source: /note="Description of Artificial Sequence: Synthetic polynucleotide"
gacatccagatgacccagagcccctccagcctgtccgcctccgtgggcgacagagtgaccatcacctgtcgggcctcccagtccatctccaactacctgaactggtatcagcagaagcccggcaaggcccctaagctgctgatctacgccgcctccaacctgcagtccggcgtgccctccagattctccggctctggctccggcaccgacttcaccctgaccatctccagcctgcagcccgaggacttcgccacctactactgcttccagtacacccacagccccgccaccttcggccagggcaccaaagtggaaatcaag

SEQ ID NO: 313 - protein, 214 aa, Artificial Sequence
  source: /note="Description of Artificial Sequence: Synthetic polypeptide"
DIQMTQSPSSLSASVGDRVTITCRASQSISNYLNWYQQKPGKAPKLLIYAASNLQSGVPSRFSGSGSGTDFTLTISSLQPEDFATYYCFQYTHSPATFGQGTKVEIKRTVAAPSVFIFPPSDEQLKSGTASVVCLLNNFYPREAKVQWKVDNALQSGNSQESVTEQDSKDSTYSLSSTLTLSKADYEKHKVYACEVTHQGLSSPVTKSFNRGEC

SEQ ID NO: 314 - DNA, 642 bp, Artificial Sequence
  source: /note="Description of Artificial Sequence: Synthetic polynucleotide"
gacatccagatgacccagagcccctccagcctgtccgcctccgtgggcgacagagtgaccatcacctgtcgggcctcccagtccatctccaactacctgaactggtatcagcagaagcccggcaaggcccctaagctgctgatctacgccgcctccaacctgcagtccggcgtgccctccagattctccggctctggctccggcaccgacttcaccctgaccatctccagcctgcagcccgaggacttcgccacctactactgcttccagtacacccacagccccgccaccttcggccagggcaccaaagtggaaatcaagcgtacggtggccgctcccagcgtgttcatcttcccccccagcgacgagcagctgaagagcggcaccgccagcgtggtgtgcctgctgaacaacttctacccccgggaggccaaggtgcagtggaaggtggacaacgccctgcagagcggcaacagccaggagagcgtcaccgagcaggacagcaaggactccacctacagcctgagcagcaccctgaccctgagcaaggccgactacgagaagcataaggtgtacgcctgcgaggtgacccaccagggcctgtccagccccgtgaccaagagcttcaacaggggcgagtgc

SEQ ID NO: 315 - protein, 10 aa, Artificial Sequence
  source: /note="Description of Artificial Sequence: Synthetic peptide"
GYTFTNYYVH

SEQ ID NO: 316 - protein, 17 aa, Artificial Sequence
  source: /note="Description of Artificial Sequence: Synthetic peptide"
WINPYSGNTNYAQKFQG

SEQ ID NO: 317 - protein, 13 aa, Artificial Sequence
  source: /note="Description of Artificial Sequence: Synthetic peptide"
GASSIRMSYYLDV

SEQ ID NO: 318 - protein, 5 aa, Artificial Sequence
  source: /note="Description of Artificial Sequence: Synthetic peptide"
NYYVH

SEQ ID NO: 319 - protein, 17 aa, Artificial Sequence
  source: /note="Description of Artificial Sequence: Synthetic peptide"
WINPYSGNTNYAQKFQG

SEQ ID NO: 320 - protein, 13 aa, Artificial Sequence
  source: /note="Description of Artificial Sequence: Synthetic peptide"
GASSIRMSYYLDV

SEQ ID NO: 321 - protein, 7 aa, Artificial Sequence
  source: /note="Description of Artificial Sequence: Synthetic peptide"
GYTFTNY

SEQ ID NO: 322 - protein, 6 aa, Artificial Sequence
  source: /note="Description of Artificial Sequence: Synthetic peptide"
NPYSGN

SEQ ID NO: 323 - protein, 13 aa, Artificial Sequence
  source: /note="Description of Artificial Sequence: Synthetic peptide"
GASSIRMSYYLDV

SEQ ID NO: 324 - protein, 8 aa, Artificial Sequence
  source: /note="Description of Artificial Sequence: Synthetic peptide"
GYTFTNYY

SEQ ID NO: 325 - protein, 8 aa, Artificial Sequence
  source: /note="Description of Artificial Sequence: Synthetic peptide"
INPYSGNT

SEQ ID NO: 326 - protein, 15 aa, Artificial Sequence
  source: /note="Description of Artificial Sequence: Synthetic peptide"
ARGASSIRMSYYLDV

SEQ ID NO: 327 - protein, 122 aa, Artificial Sequence
  source: /note="Description of Artificial Sequence: Synthetic polypeptide"
QVQLVQSGAEVKKPGASVKVSCKASGYTFTNYYVHWVRQAPGQGLEWMGWINPYSGNTNYAQKFQGRVTMTRDTSISTAYMELSRLRSEDTAVYYCARGASSIRMSYYLDVWGQGTLVTVSS

SEQ ID NO: 328 - DNA, 366 bp, Artificial Sequence
  source: /note="Description of Artificial Sequence: Synthetic polynucleotide"
caagtgcagctggtgcagtctggcgctgaagtgaagaaacctggcgcctccgtgaaagtgtcctgcaaggcctccggctacaccttcaccaactactacgtgcactgggtccgacaggccccaggccagggcctggagtggatgggctggatcaacccctactccggcaacaccaactacgcccagaaattccagggcagagtgaccatgacccgggacacctccatctccaccgcctacatggaactgtcccggctgcggagcgaggacaccgccgtgtactactgtgccagaggcgcctcctccatccggatgtcctactacctggacgtgtggggccagggcaccctggtcaccgtgtcctct

SEQ ID NO: 329 - protein, 225 aa, Artificial Sequence
  source: /note="Description of Artificial Sequence: Synthetic polypeptide"
QVQLVQSGAEVKKPGASVKVSCKASGYTFTNYYVHWVRQAPGQGLEWMGWINPYSGNTNYAQKFQGRVTMTRDTSISTAYMELSRLRSEDTAVYYCARGASSIRMSYYLDVWGQGTLVTVSSASTKGPSVFPLAPSSKSTSGGTAALGCLVKDYFPEPVTVSWNSGALTSGVHTFPAVLQSSGLYSLSSVVTVPSSSLGTQTYICNVNHKPSNTKVDKRVEPKSC

SEQ ID NO: 330 - DNA, 675 bp, Artificial Sequence
  source: /note="Description of Artificial Sequence: Synthetic polynucleotide"
caagtgcagctggtgcagtctggcgctgaagtgaagaaacctggcgcctccgtgaaagtgtcctgcaaggcctccggctacaccttcaccaactactacgtgcactgggtccgacaggccccaggccagggcctggagtggatgggctggatcaacccctactccggcaacaccaactacgcccagaaattccagggcagagtgaccatgacccgggacacctccatctccaccgcctacatggaactgtcccggctgcggagcgaggacaccgccgtgtactactgtgccagaggcgcctcctccatccggatgtcctactacctggacgtgtggggccagggcaccctggtcaccgtgtcctctgctagcaccaagggcccctccgtgttccctctggccccttccagcaagtctacctctggcggcaccgctgctctgggctgcctggtgaaggactacttccctgagcctgtgacagtgtcctggaactctggcgccctgacctccggcgtgcacaccttccctgccgtgctgcagtcctccggcctgtactccctgtcctccgtggtgacagtgccttcctccagcctgggcacccagacctatatctgcaacgtgaaccacaagccttccaacaccaaggtggacaagcgggtggagcctaagtcatgc

SEQ ID NO: 331 - protein, 11 aa, Artificial Sequence
  source: /note="Description of Artificial Sequence: Synthetic peptide"
RASQSISNYLN

SEQ ID NO: 332 - protein, 7 aa, Artificial Sequence
  source: /note="Description of Artificial Sequence: Synthetic peptide"
AASNLQS

SEQ ID NO: 333 - protein, 9 aa, Artificial Sequence
  source: /note="Description of Artificial Sequence: Synthetic peptide"
FQYTHSPAT

SEQ ID NO: 334 - protein, 11 aa, Artificial Sequence
  source: /note="Description of Artificial Sequence: Synthetic peptide"
RASQSISNYLN

SEQ ID NO: 335 - protein, 7 aa, Artificial Sequence
  source: /note="Description of Artificial Sequence: Synthetic peptide"
AASNLQS

SEQ ID NO: 336 - protein, 9 aa, Artificial Sequence
  source: /note="Description of Artificial Sequence: Synthetic peptide"
FQYTHSPAT

SEQ ID NO: 337 - protein, 7 aa, Artificial Sequence
  source: /note="Description of Artificial Sequence: Synthetic peptide"
SQSISNY

SEQ ID NO: 338 - protein, 3 aa, Artificial Sequence
  source: /note="Description of Artificial Sequence: Synthetic peptide"
AAS

SEQ ID NO: 339 - protein, 6 aa, Artificial Sequence
  source: /note="Description of Artificial Sequence: Synthetic peptide"
YTHSPA

SEQ ID NO: 340 - protein, 6 aa, Artificial Sequence
  source: /note="Description of Artificial Sequence: Synthetic peptide"
QSISNY

SEQ ID NO: 341 - protein, 3 aa, Artificial Sequence
  source: /note="Description of Artificial Sequence: Synthetic peptide"
AAS

SEQ ID NO: 342 - protein, 9 aa, Artificial Sequence
  source: /note="Description of Artificial Sequence: Synthetic peptide"
FQYTHSPAT

SEQ ID NO: 343 - protein, 107 aa, Artificial Sequence; identical to SEQ ID NO: 311
  source: /note="Description of Artificial Sequence: Synthetic polypeptide"

SEQ ID NO: 344 - DNA, 321 bp, Artificial Sequence; identical to SEQ ID NO: 312
  source: /note="Description of Artificial Sequence: Synthetic polynucleotide"

SEQ ID NO: 345 - protein, 214 aa, Artificial Sequence; identical to SEQ ID NO: 313
  source: /note="Description of Artificial Sequence: Synthetic polypeptide"

SEQ ID NO: 346 - DNA, 642 bp, Artificial Sequence; identical to SEQ ID NO: 314
  source: /note="Description of Artificial Sequence: Synthetic polynucleotide"

SEQ ID NO: 347 - protein, 10 aa, Artificial Sequence
  source: /note="Description of Artificial Sequence: Synthetic peptide"
  MOD_RES (5)..(5): Any amino acid
  source: /note="See specification as filed for detailed description of substitutions and preferred embodiments"
GFTFXSAAVH

SEQ ID NO: 348 - protein, 19 aa, Artificial Sequence
  source: /note="Description of Artificial Sequence: Synthetic peptide"
  MOD_RES (7)..(7): Any amino acid
  source: /note="See specification as filed for detailed description of substitutions and preferred embodiments"
RIKSKAXGGTTDYAAPVKG

SEQ ID NO: 349 - protein, 19 aa, Artificial Sequence
  source: /note="Description of Artificial Sequence: Synthetic peptide"
  MOD_RES (6)..(7): Any amino acid
  source: /note="See specification as filed for detailed description of substitutions and preferred embodiments"
RIKSKXXGGTTDYAAPVKG

SEQ ID NO: 350 - protein, 18 aa, Artificial Sequence
  source: /note="Description of Artificial Sequence: Synthetic peptide"
DSPSISSYSIPYFSGMDV

SEQ ID NO: 351 - protein, 11 aa, Artificial Sequence
  source: /note="Description of Artificial Sequence: Synthetic peptide"
RASQGIRAWLN

SEQ ID NO: 352 - protein, 11 aa, Artificial Sequence
  source: /note="Description of Artificial Sequence: Synthetic peptide"
  MOD_RES (5)..(5): Any amino acid
  MOD_RES (7)..(9): Any amino acid
  source: /note="See specification as filed for detailed description of substitutions and preferred embodiments"
RASQXIXXXLN

SEQ ID NO: 353 - protein, 7 aa, Artificial Sequence
  source: /note="Description of Artificial Sequence: Synthetic peptide"
AASSLQS

SEQ ID NO: 354 - protein, 9 aa, Artificial Sequence
  source: /note="Description of Artificial Sequence: Synthetic peptide"
HQYITHPPT

SEQ ID NO: 355 - protein, 9 aa, Artificial Sequence
  source: /note="Description of Artificial Sequence: Synthetic peptide"
  MOD_RES (5)..(6): Any amino acid
  MOD_RES (8)..(8): Any amino acid
  source: /note="See specification as filed for detailed description of substitutions and preferred embodiments"
HQYIXXPXT

SEQ ID NO: 356 - protein, 5 aa, Artificial Sequence
  source: /note="Description of Artificial Sequence: Synthetic peptide"
SAAVH

SEQ ID NO: 357 - protein, 19 aa, Artificial Sequence
  source: /note="Description of Artificial Sequence: Synthetic peptide"
  MOD_RES (7)..(8): Any amino acid
  source: /note="See specification as filed for detailed description of substitutions and preferred embodiments"
RIKSKAXXGTTDYAAPVKG

SEQ ID NO: 358 - protein, 19 aa, Artificial Sequence
  source: /note="Description of Artificial Sequence: Synthetic peptide"
  MOD_RES (6)..(8): Any amino acid
  source: /note="See specification as filed for detailed description of substitutions and preferred embodiments"
RIKSKXXXGTTDYAAPVKG

SEQ ID NO: 359 - protein, 7 aa, Artificial Sequence
  source: /note="Description of Artificial Sequence: Synthetic peptide"
  MOD_RES (4)..(4): Any amino acid
AASXLQS

SEQ ID NO: 360 - protein, 452 aa, Artificial Sequence
  source: /note="Description of Artificial Sequence: Synthetic polypeptide"
QVQLLESGGGLVQPGGSLRLSCAASGFTFSTAAMSWVRQAPGKGLEWVSGISGSGSSTYYADSVKGRFTISRDNSKNTLYLQMNSLRAEDTAVYYCARELSYLYSGYYFDYWGQGTLVTVSSASTKGPSVFPLAPSSKSTSGGTAALGCLVKDYFPEPVTVSWNSGALTSGVHTFPAVLQSSGLYSLSSVVTVPSSSLGTQTYICNVNHKPSNTKVDKRVEPKSCDKTHTCPPCPAPEAAGGPSVFLFPPKPKDTLMISRTPEVTCVVVDVSHEDPEVKFNWYVDGVEVHNAKTKPREEQYNSTYRVVSVLTVLHQDWLNGKEYKCKVSNKALPAPIEKTISKAKGQPREPQVYTLPPSREEMTKNQVSLTCLVKGFYPSDIAVEWESNGQPENNYKTTPPVLDSDGSFFLYSKLTVDKSRWQQGNVFSCSVMHEALHNHYTQKSLSLSPGK

SEQ ID NO: 361 - DNA, 1356 bp, Artificial Sequence
  source: /note="Description of Artificial Sequence: Synthetic polynucleotide"
caggtgcaattgctggaaagcggcggtggcctggtgcagccgggtggcagcctgcgtctgagctgcgcggcgtccggattcaccttttctactgctgctatgtcttgggtgcgccaggccccgggcaaaggtctcgagtgggtttccggtatctctggttctggttcttctacctactatgcggatagcgtgaaaggccgctttaccatcagccgcgataattcgaaaaacaccctgtatctgcaaatgaacagcctgcgtgcggaagatacggccgtgtattattgcgcgcgtgaactgtcttacctgtactctggttactacttcgattactggggccaaggcaccctggtgactgttagctcagcctccaccaagggtccatcggtcttccccctggcaccctcctccaagagcacctctgggggcacagcggccctgggctgcctggtcaaggactacttccccgaaccggtgacggtgtcgtggaactcaggcgccctgaccagcggcgtgcacaccttcccggctgtcctacagtcctcaggactctactccctcagcagcgtggtgaccgtgccctccagcagcttgggcacccagacctacatctgcaacgtgaatcacaagcccagcaacaccaaggtggacaagagagttgagcccaaatcttgtgacaaaactcacacatgcccaccgtgcccagcacctgaagcagcggggggaccgtcagtcttcctcttccccccaaaacccaaggacaccctcatgatctcccggacccctgaggtcacatgcgtggtggtggacgtgagccacgaagaccctgaggtcaagttcaactggtacgtggacggcgtggaggtgcataatgccaagacaaagccgcgggaggagcagtacaacagcacgtaccgggtggtcagcgtcctcaccgtcctgcaccaggactggctgaatggcaaggagtacaagtgcaaggtctccaacaaagccctcccagcccccatcgagaaaaccatctccaaagccaaagggcagccccgagaaccacaggtgtacaccctgcccccatcccgggaggagatgaccaagaaccaggtcagcctgacctgcctggtcaaaggcttctatcccagcgacatcgccgtggagtgggagagcaatgggcagccggagaacaactacaagaccacgcctcccgtgctggactccgacggctccttcttcctctacagcaagctcaccgtggacaagagcaggtggcagcaggggaacgtcttctcatgctccgtgatgcatgaggctctgcacaaccactacacgcagaagagcctctccctgtctccgggtaaa

SEQ ID NO: 362 - protein, 110 aa, Artificial Sequence
  source: /note="Description of Artificial Sequence: Synthetic polypeptide"
DIVLTQPPSVSGAPGQRVTISCSGSSSNIGSNDVSWYQQLPGTAPKLLIYKNYNRPSGVPDRFSGSKSGTSASLAITGLQAEDEADYYCSAWDQRQFDVVFGGGTKLTVL

SEQ ID NO: 363 - DNA, 330 bp, Artificial Sequence
  source: /note="Description of Artificial Sequence: Synthetic polynucleotide"
gatatcgtgctgacccagccgccgagcgtgagcggtgcaccgggccagcgcgtgaccattagctgtagcggcagcagcagcaacattggttctaacgacgtgtcttggtaccagcagctgccgggcacggcgccgaaactgctgatctacaaaaactacaaccgcccgagcggcgtgccggatcgctttagcggatccaaaagcggcaccagcgccagcctggcgattaccggcctgcaagcagaagacgaagcggattattactgctctgcttgggaccagcgtcagttcgacgttgtgtttggcggcggcacgaagttaaccgtccta

SEQ ID NO: 364 - protein, 216 aa, Artificial Sequence
  source: /note="Description of Artificial Sequence: Synthetic polypeptide"
DIVLTQPPSVSGAPGQRVTISCSGSSSNIGSNDVSWYQQLPGTAPKLLIYKNYNRPSGVPDRFSGSKSGTSASLAITGLQAEDEADYYCSAWDQRQFDVVFGGGTKLTVLGQPKAAPSVTLFPPSSEELQANKATLVCLISDFYPGAVTVAWKADSSPVKAGVETTTPSKQSNNKYAASSYLSLTPEQWKSHRSYSCQVTHEGSTVEKTVAPTECS

SEQ ID NO: 365 - DNA, 648 bp, Artificial Sequence
  source: /note="Description of Artificial Sequence: Synthetic polynucleotide"
gatatcgtgctgacccagccgccgagcgtgagcggtgcaccgggccagcgcgtgaccattagctgtagcggcagcagcagcaacattggttctaacgacgtgtcttggtaccagcagctgccgggcacggcgccgaaactgctgatctacaaaaactacaaccgcccgagcggcgtgccggatcgctttagcggatccaaaagcggcaccagcgccagcctggcgattaccggcctgcaagcagaagacgaagcggattattactgctctgcttgggaccagcgtcagttcgacgttgtgtttggcggcggcacgaagttaaccgtcctaggtcagcccaaggctgccccctcggtcactctgttcccgccctcctctgaggagcttcaagccaacaaggccacactggtgtgtctcataagtgacttctacccgggagccgtgacagtggcctggaaggcagatagcagccccgtcaaggcgggagtggagaccaccacaccctccaaacaaagcaacaacaagtacgcggccagcagctatctgagcctgacgcctgagcagtggaagtcccacagaagctacagctgccaggtcacgcatgaagggagcaccgtggagaagacagtggcccctacagaatgttca

SEQ ID NO: 366 - protein, 17 aa, Artificial Sequence
  source: /note="Description of Artificial Sequence: Synthetic peptide"
TIDSWGDDTDYADSVKG

SEQ ID NO: 367 - protein, 6 aa, Artificial Sequence
  source: /note="Description of Artificial Sequence: Synthetic peptide"
DSWGDD

SEQ ID NO: 368 - protein, 8 aa, Artificial Sequence
  source: /note="Description of Artificial Sequence: Synthetic peptide"
IDSWGDDT

SEQ ID NO: 369 - protein, 122 aa, Artificial Sequence
  source: /note="Description of Artificial Sequence: Synthetic polypeptide"
QVQLLESGGGLVQPGGSLRLSCAASGFTFSTAAMSWVRQAPGKGLEWVSTIDSWGDDTDYADSVKGRFTISRDNSKNTLYLQMNSLRAEDTAVYYCARELSYLYSGYYFDYWGQGTLVTVSS

SEQ ID NO: 370 - DNA, 366 bp, Artificial Sequence
  source: /note="Description of Artificial Sequence: Synthetic polynucleotide"
caggtgcaattgctggaaagcggcggtggcctggtgcagccgggtggcagcctgcgtctgagctgcgcggcgtccggattcaccttttctactgctgctatgtcttgggtgcgccaggccccgggcaaaggtctcgagtgggtttccactatcgactcttggggcgacgacactgactatgcggatagcgtgaaaggccgctttaccatcagccgcgataattcgaaaaacaccctgtatctgcaaatgaacagcctgcgtgcggaagatacggccgtgtattattgcgcgcgtgaactgtcttacctgtactctggttactacttcgattactggggccaaggcaccctggtgactgttagctca

SEQ ID NO: 371 - protein, 452 aa, Artificial Sequence
  source: /note="Description of Artificial Sequence: Synthetic polypeptide"
QVQLLESGGGLVQPGGSLRLSCAASGFTFSTAAMSWVRQAPGKGLEWVSTIDSWGDDTDYADSVKGRFTISRDNSKNTLYLQMNSLRAEDTAVYYCARELSYLYSGYYFDYWGQGTLVTVSSASTKGPSVFPLAPSSKSTSGGTAALGCLVKDYFPEPVTVSWNSGALTSGVHTFPAVLQSSGLYSLSSVVTVPSSSLGTQTYICNVNHKPSNTKVDKRVEPKSCDKTHTCPPCPAPEAAGGPSVFLFPPKPKDTLMISRTPEVTCVVVDVSHEDPEVKFNWYVDGVEVHNAKTKPREEQYNSTYRVVSVLTVLHQDWLNGKEYKCKVSNKALPAPIEKTISKAKGQPREPQVYTLPPSREEMTKNQVSLTCLVKGFYPSDIAVEWESNGQPENNYKTTPPVLDSDGSFFLYSKLTVDKSRWQQGNVFSCSVMHEALHNHYTQKSLSLSPGK

SEQ ID NO: 372 - protein, 17 aa, Artificial Sequence
  source: /note="Description of Artificial Sequence: Synthetic peptide"
SIEYYDTDTHYADSVKG

SEQ ID NO: 373 - protein, 6 aa, Artificial Sequence
  source: /note="Description of Artificial Sequence: Synthetic peptide"
EYYDTD

SEQ ID NO: 374 - protein, 8 aa, Artificial Sequence
  source: /note="Description of Artificial Sequence: Synthetic peptide"
IEYYDTDT

SEQ ID NO: 375 - protein, 122 aa, Artificial Sequence
  source: /note="Description of Artificial Sequence: Synthetic polypeptide"
QVQLLESGGGLVQPGGSLRLSCAASGFTFSTAAMSWVRQAPGKGLEWVSSIEYYDTDTHYADSVKGRFTISRDNSKNTLYLQMNSLRAEDTAVYYCARELSYLYSGYYFDYWGQGTLVTVSS

SEQ ID NO: 376 - DNA, 366 bp, Artificial Sequence
  source: /note="Description of Artificial Sequence: Synthetic polynucleotide"
caggtgcaattgctggaaagcggcggtggcctggtgcagccgggtggcagcctgcgtctgagctgcgcggcgtccggattcaccttttctactgctgctatgtcttgggtgcgccaggccccgggcaaaggtctcgagtgggtttcctctatcgaatactacgacactgacactcattatgcggatagcgtgaaaggccgctttaccatcagccgcgataattcgaaaaacaccctgtatctgcaaatgaacagcctgcgtgcggaagatacggccgtgtattattgcgcgcgtgaactgtcttacctgtactctggttactacttcgattactggggccaaggcaccctggtgactgttagctca

SEQ ID NO: 377 - protein, 452 aa, Artificial Sequence
  source: /note="Description of Artificial Sequence: Synthetic polypeptide"
QVQLLESGGGLVQPGGSLRLSCAASGFTFSTAAMSWVRQAPGKGLEWVSSIEYYDTDTHYADSVKGRFTISRDNSKNTLYLQMNSLRAEDTAVYYCARELSYLYSGYYFDYWGQGTLVTVSSASTKGPSVFPLAPSSKSTSGGTAALGCLVKDYFPEPVTVSWNSGALTSGVHTFPAVLQSSGLYSLSSVVTVPSSSLGTQTYICNVNHKPSNTKVDKRVEPKSCDKTHTCPPCPAPEAAGGPSVFLFPPKPKDTLMISRTPEVTCVVVDVSHEDPEVKFNWYVDGVEVHNAKTKPREEQYNSTYRVVSVLTVLHQDWLNGKEYKCKVSNKALPAPIEKTISKAKGQPREPQVYTLPPSREEMTKNQVSLTCLVKGFYPSDIAVEWESNGQPENNYKTTPPVLDSDGSFFLYSKLTVDKSRWQQGNVFSCSVMHEALHNHYTQKSLSLSPGK

SEQ ID NO: 378 - DNA, 1356 bp, Artificial Sequence
  source: /note="Description of Artificial Sequence: Synthetic polynucleotide"
caggtgcaattgctggaaagcggcggtggcctggtgcagccgggtggcagcctgcgtctgagctgcgcggcgtccggattcaccttttctactgctgctatgtcttgggtgcgccaggccccgggcaaaggtctcgagtgggtttcctctatcgaatactacgacactgacactcattatgcggatagcgtgaaaggccgctttaccatcagccgcgataattcgaaaaacaccctgtatctgcaaatgaacagcctgcgtgcggaagatacggccgtgtattattgcgcgcgtgaactgtcttacctgtactctggttactacttcgattactggggccaaggcaccctggtgactgttagctcagcctccaccaagggtccatcggtcttccccctggcaccctcctccaagagcacctctgggggcacagcggccctgggctgcctggtcaaggactacttccccgaaccggtgacggtgtcgtggaactcaggcgccctgaccagcggcgtgcacaccttcccggctgtcctacagtcctcaggactctactccctcagcagcgtggtgaccgtgccctccagcagcttgggcacccagacctacatctgcaacgtgaatcacaagcccagcaacaccaaggtggacaagagagttgagcccaaatcttgtgacaaaactcacacatgcccaccgtgcccagcacctgaagcagcggggggaccgtcagtcttcctcttccccccaaaacccaaggacaccctcatgatctcccggacccctgaggtcacatgcgtggtggtggacgtgagccacgaagaccctgaggtcaagttcaactggtacgtggacggcgtggaggtgcataatgccaagacaaagccgcgggaggagcagtacaacagcacgtaccgggtggtcagcgtcctcaccgtcctgcaccaggactggctgaatggcaaggagtacaagtgcaaggtctccaacaaagccctcccagcccccatcgagaaaaccatctccaaagccaaagggcagccccgagaaccacaggtgtacaccctgcccccatcccgggaggagatgaccaagaaccaggtcagcctgacctgcctggtcaaaggcttctatcccagcgacatcgccgtggagtgggagagcaatgggcagccggagaacaactacaagaccacgcctcccgtgctggactccgacggctccttcttcctctacagcaagctcaccgtggacaagagcaggtggcagcaggggaacgtcttctcatgctccgtgatgcatgaggctctgcacaaccactacacgcagaagagcctctccctgtctccgggtaaa

SEQ ID NO: 379 - protein, 17 aa, Artificial Sequence
  source: /note="Description of Artificial Sequence: Synthetic peptide"
TIEYSSQETYYADSVKG

SEQ ID NO: 380 - protein, 6 aa, Artificial Sequence
  source: /note="Description of Artificial Sequence: Synthetic peptide"
EYSSQE

SEQ ID NO: 381 - protein, 8 aa, Artificial Sequence
  source: /note="Description of Artificial Sequence: Synthetic peptide"
IEYSSQET

SEQ ID NO: 382 - protein, 122 aa, Artificial Sequence
  source: /note="Description of Artificial Sequence: Synthetic polypeptide"
QVQLLESGGGLVQPGGSLRLSCAASGFTFSTAAMSWVRQAPGKGLEWVSTIEYSSQETYYADSVKGRFTISRDNSKNTLYLQMNSLRAEDTAVYYCARELSYLYSGYYFDYWGQGTLVTVSS

SEQ ID NO: 383 - DNA, 366 bp, Artificial Sequence
  source: /note="Description of Artificial Sequence: Synthetic polynucleotide"
caggtgcaattgctggaaagcggcggtggcctggtgcagccgggtggcagcctgcgtctgagctgcgcggcgtccggattcaccttttctactgctgctatgtcttgggtgcgccaggccccgggcaaaggtctcgagtgggtttccactatcgaatactctagccaggaaacttactatgcggatagcgtgaaaggccgctttaccatcagccgcgataattcgaaaaacaccctgtatctgcaaatgaacagcctgcgtgcggaagatacggccgtgtattattgcgcgcgtgaactgtcttacctgtactctggttactacttcgattactggggccaaggcaccctggtgactgttagctca

SEQ ID NO: 384 - protein, 452 aa, Artificial Sequence
  source: /note="Description of Artificial Sequence: Synthetic polypeptide"
QVQLLESGGGLVQPGGSLRLSCAASGFTFSTAAMSWVRQAPGKGLEWVSTIEYSSQETYYADSVKGRFTISRDNSKNTLYLQMNSLRAEDTAVYYCARELSYLYSGYYFDYWGQGTLVTVSSASTKGPSVFPLAPSSKSTSGGTAALGCLVKDYFPEPVTVSWNSGALTSGVHTFPAVLQSSGLYSLSSVVTVPSSSLGTQTYICNVNHKPSNTKVDKRVEPKSCDKTHTCPPCPAPEAAGGPSVFLFPPKPKDTLMISRTPEVTCVVVDVSHEDPEVKFNWYVDGVEVHNAKTKPREEQYNSTYRVVSVLTVLHQDWLNGKEYKCKVSNKALPAPIEKTISKAKGQPREPQVYTLPPSREEMTKNQVSLTCLVKGFYPSDIAVEWESNGQPENNYKTTPPVLDSDGSFFLYSKLTVDKSRWQQGNVFSCSVMHEALHNHYTQKSLSLSPGK

SEQ ID NO: 385 - DNA, 1356 bp, Artificial Sequence
  source: /note="Description of Artificial Sequence: Synthetic polynucleotide"
caggtgcaattgctggaaagcggcggtggcctggtgcagccgggtggcagcctgcgtctgagctgcgcggcgtccggattcaccttttctactgctgctatgtcttgggtgcgccaggccccgggcaaaggtctcgagtgggtttccactatcgaatactctagccaggaaacttactatgcggatagcgtgaaaggccgctttaccatcagccgcgataattcgaaaaacaccctgtatctgcaaatgaacagcctgcgtgcggaagatacggccgtgtattattgcgcgcgtgaactgtcttacctgtactctggttactacttcgattactggggccaaggcaccctggtgactgttagctcagcctccaccaagggtccatcggtcttccccctggcaccctcctccaagagcacctctgggggcacagcggccctgggctgcctggtcaaggactacttccccgaaccggtgacggtgtcgtggaactcaggcgccctgaccagcggcgtgcacaccttcccggctgtcctacagtcctcaggactctactccctcagcagcgtggtgaccgtgccctccagcagcttgggcacccagacctacatctgcaacgtgaatcacaagcccagcaacaccaaggtggacaagagagttgagcccaaatcttgtgacaaaactcacacatgcccaccgtgcccagcacctgaagcagcggggggaccgtcagtcttcctcttccccccaaaacccaaggacaccctcatgatctcccggacccctgaggtcacatgcgtggtggtggacgtgagccacgaagaccctgaggtcaagttcaactggtacgtggacggcgtggaggtgcataatgccaagacaaagccgcgggaggagcagtacaacagcacgtaccgggtggtcagcgtcctcaccgtcctgcaccaggactggctgaatggcaaggagtacaagtgcaaggtctccaacaaagccctcccagcccccatcgagaaaaccatctccaaagccaaagggcagccccgagaaccacaggtgtacaccctgcccccatcccgggaggagatgaccaagaaccaggtcagcctgacctgcctggtcaaaggcttctatcccagcgacatcgccgtggagtgggagagcaatgggcagccggagaacaactacaagaccacgcctcccgtgctggactccgacggctccttcttcctctacagcaagctcaccgtggacaagagcaggtggcagcaggggaacgtcttctcatgctccgtgatgcatgaggctctgcacaaccactacacgcagaagagcctctccctgtctccgggtaaa

SEQ ID NO: 386 - protein, 110 aa, Artificial Sequence
  source: /note="Description of Artificial Sequence: Synthetic polypeptide"
QSVLTQPPSVSGAPGQRVTISCSGSSSNIGSNDVSWYQQLPGTAPKLLIYKNYNRPSGVPDRFSGSKSGTSASLAITGLQAEDEADYYCSAWDQRQFDVVFGGGTKLTVL

SEQ ID NO: 387 - DNA, 330 bp, Artificial Sequence
  source: /note="Description of Artificial Sequence: Synthetic polynucleotide"
cagagcgtgctgacacagcctccctccgtgtctggcgcccctggccagagagtgaccatctcctgctccggctcctcctccaacatcggctccaacgacgtgtcctggtatcagcagctgcccggcaccgcccctaagctgctgatctacaagaactacaaccggccctccggcgtgcccgaccggttctctggctccaagtctggcacctccgcctccctggctatcaccggcctgcaggctgaggacgaggccgactactactgctccgcctgggaccagcggcagttcgacgtggtgttcggcggaggcaccaagctgaccgtgctg

SEQ ID NO: 388 - protein, 216 aa, Artificial Sequence
  source: /note="Description of Artificial Sequence: Synthetic polypeptide"
QSVLTQPPSVSGAPGQRVTISCSGSSSNIGSNDVSWYQQLPGTAPKLLIYKNYNRPSGVPDRFSGSKSGTSASLAITGLQAEDEADYYCSAWDQRQFDVVFGGGTKLTVLGQPKAAPSVTLFPPSSEELQANKATLVCLISDFYPGAVTVAWKADSSPVKAGVETTTPSKQSNNKYAASSYLSLTPEQWKSHRSYSCQVTHEGSTVEKTVAPTECS

SEQ ID NO: 389 - DNA, 648 bp, Artificial Sequence
  source: /note="Description of Artificial Sequence: Synthetic polynucleotide"
cagagcgtgctgacacagcctccctccgtgtctggcgcccctggccagagagtgaccatctcctgctccggctcctcctccaacatcggctccaacgacgtgtcctggtatcagcagctgcccggcaccgcccctaagctgctgatctacaagaactacaaccggccctccggcgtgcccgaccggttctctggctccaagtctggcacctccgcctccctggctatcaccggcctgcaggctgaggacgaggccgactactactgctccgcctgggaccagcggcagttcgacgtggtgttcggcggaggcaccaagctgaccgtgctgggccagcctaaggctgcccccagcgtgaccctgttcccccccagcagcgaggagctgcaggccaacaaggccaccctggtgtgcctgatcagcgacttctacccaggcgccgtgaccgtggcctggaaggccgacagcagccccgtgaaggccggcgtggagaccaccacccccagcaagcagagcaacaacaagtacgccgccagcagctacctgagcctgacccccgagcagtggaagagccacaggtcctacagctgccaggtgacccacgagggcagcaccgtggaaaagaccgtggccccaaccgagtgcagc

SEQ ID NO: 390 - DNA, 366 bp, Artificial Sequence
  source: /note="Description of Artificial Sequence: Synthetic polynucleotide"
caggtgcaattgctggaaagcggcggtggcctggtgcagccgggtggcagcctgcgtctgagctgcgcggcgtccggattcaccttttctactgctgctatgtcttgggtgcgccaggccccgggcaaaggtctcgagtgggtttccggtatctctggttctggttcttctacctactatgcggatagcgtgaaaggccgctttaccatcagccgcgataattcgaaaaacaccctgtatctgcaaatgaacagcctgcgtgcggaagatacggccgtgtattattgcgcgcgtgaactgtcttacctgtactctggttactacttcgattactggggccaaggcaccctggtgactgttagctca

SEQ ID NO: 391 - DNA, 1356 bp, Artificial Sequence
  source: /note="Description of Artificial Sequence: Synthetic polynucleotide"
caggtgcaattgctggaaagcggcggtggcctggtgcagccgggtggcagcctgcgtctgagctgcgcggcgtccggattcaccttttctactgctgctatgtcttgggtgcgccaggccccgggcaaaggtctcgagtgggtttccactatcgactcttggggcgacgacactgactatgcggatagcgtgaaaggccgctttaccatcagccgcgataattcgaaaaacaccctgtatctgcaaatgaacagcctgcgtgcggaagatacggccgtgtattattgcgcgcgtgaactgtcttacctgtactctggttactacttcgattactggggccaaggcaccctggtgactgttagctcagcctccaccaagggtccatcggtcttccccctggcaccctcctccaagagcacctctgggggcacagcggccctgggctgcctggtcaaggactacttccccgaaccggtgacggtgtcgtggaactcaggcgccctgaccagcggcgtgcacaccttcccggctgtcctacagtcctcaggactctactccctcagcagcgtggtgaccgtgccctccagcagcttgggcacccagacctacatctgcaacgtgaatcacaagcccagcaacaccaaggtggacaagagagttgagcccaaatcttgtgacaaaactcacacatgcccaccgtgcccagcacctgaagcagcggggggaccgtcagtcttcctcttccccccaaaacccaaggacaccctcatgatctcccggacccctgaggtcacatgcgtggtggtggacgtgagccacgaagaccctgaggtcaagttcaactggtacgtggacggcgtggaggtgcataatgccaagacaaagccgcgggaggagcagtacaacagcacgtaccgggtggtcagcgtcctcaccgtcctgcaccaggactggctgaatggcaaggagtacaagtgcaaggtctccaacaaagccctcccagcccccatcgagaaaaccatctccaaagccaaagggcagccccgagaaccacaggtgtacaccctgcccccatcccgggaggagatgaccaagaaccaggtcagcctgacctgcctggtcaaaggcttctatcccagcgacatcgccgtggagtgggagagcaatgggcagccggagaacaactacaagaccacgcctcccgtgctggactccgacggctccttcttcctctacagcaagctcaccgtggacaagagcaggtggcagcaggggaacgtcttctcatgctccgtgatgcatgaggctctgcacaaccactacacgcagaagagcctctccctgtctccgggtaaa

SEQ ID NO: 392 - DNA, 366 bp, Artificial Sequence
  source: /note="Description of Artificial Sequence: Synthetic polynucleotide"
caagtgcagctgcttgaatctggcggcggactggtgcagcctggcggctccctgagactgtcttgcgccgcctccggcttcaccttctccaccgccgctatgtcctgggtccgacaggctcccggcaagggcctggaatgggtgtccaccattgagtactccagccaggaaacctactacgccgactccgtgaagggccggttcaccatctcccgggacaactccaagaacaccctgtacctgcagatgaactccctgcgggccgaggacaccgccgtgtactactgcgccagagagctgtcctacctgtactccggctactacttcgactactggggccagggcaccctggtcaccgtgtcctct

SEQ ID NO: 393 - DNA, 1356 bp, Artificial Sequence
  source: /note="Description of Artificial Sequence: Synthetic polynucleotide"
caagtgcagctgcttgaatctggcggcggactggtgcagcctggcggctccctgagactgtcttgcgccgcctccggcttcaccttctccaccgccgctatgtcctgggtccgacaggctcccggcaagggcctggaatgggtgtccaccattgagtactccagccaggaaacctactacgccgactccgtgaagggccggttcaccatctcccgggacaactccaagaacaccctgtacctgcagatgaactccctgcgggccgaggacaccgccgtgtactactgcgccagagagctgtcctacctgtactccggctactacttcgactactggggccagggcaccctggtcaccgtgtcctctgctagcaccaagggcccctccgtgttccctctggccccttccagcaagtctacctccggcggcacagctgctctgggctgcctggtcaaggactacttccctgagcctgtgacagtgtcctggaactctggcgccctgacctctggcgtgcacaccttccctgccgtgctgcagtcctccggcctgtactccctgtcctccgtggtcacagtgccttcaagcagcctgggcacccagacctatatctgcaacgtgaaccacaagccttccaacaccaaggtggacaagcgggtggagcctaagtcctgcgacaagacccacacctgtcctccctgccctgctcctgaagctgctggcggcccttctgtgttcctgttccctccaaagcccaaggacaccctgatgatctcccggacccctgaagtgacctgcgtggtggtggacgtgtcccacgaggatcctgaagtgaagttcaattggtacgtggacggcgtggaggtgcacaacgccaagaccaagcctcgggaggaacagtacaactccacctaccgggtggtgtccgtgctgaccgtgctgcaccaggactggctgaacggcaaagagtacaagtgcaaagtctccaacaaggccctgcctgcccctatcgaaaagacaatctccaaggccaagggccagcctagggaaccccaggtgtacaccctgccacccagccgggaggaaatgaccaagaaccaggtgtccctgacctgtctggtcaagggcttctacccttccgatatcgccgtggagtgggagtctaacggccagcctgagaacaactacaagaccacccctcctgtgctggactccgacggctccttcttcctgtactccaaactgaccgtggacaagtcccggtggcagcagggcaacgtgttctcctgctccgtgatgcacgaggccctgcacaaccactacacccagaagtccctgtccctgtctcccggcaag

SEQ ID NO: 394 - protein, 6 aa, Artificial Sequence
  source: /note="Description of Artificial Sequence: Synthetic 6xHis tag"
HHHHHH